European Patent Application EP 4 317 456 A2, published February 7, 2024. Title: Piezo Type Mechanosensitive Ion Channel Component 1 (PIEZO1) Variants And Uses Thereof. Applicant: Regeneron Pharmaceuticals, Inc. The sequence listing filed with the application follows.

SEQUENCE LISTING (4 sequences)

SEQ ID NO: 1 - DNA, 69883 bp, Homo sapiens
  source 1..69883: mol_type = other DNA
gggagccgccgtccggcccagctcggccccagtgagccgagcgctgcgctccgccgaggggcagggcggtcgcctgagcgagcgcgggcccgggacgtcggcaccggcggggcggccgaaggagaaggaggaagaggagaaggcggcgcgcgggtccccgcgggtcagccatggcgcgccggccccggggcccccgcaccgccccatagcgccgcggcgtccgctcggtctgggccgggccctgggccctccagccatggagccgcacgtgctcggcgcggtcctgtactggctgctgctgccctgcgcgctgctggctggtgagtggggggcgggcgcctgggggcgacgggagggggctgcgtctcggctccccacggcctggacaccggacgacgccggccggggcgagggctgcgggcgagcgggcgcggaaattcccagggacgcgcgacccgggcgcccgcattcctgaagcatgagcgcgccaggcggcggcggggctcctgtcccagggccgggctggaagggcggcggcggctgggggagacggcaccgcgtgcccacgggggcggtcgagcgagcgccgggcatagcgcggctggcgtctccgccggggcgctgcggagaggaggccgccgggcgaggcggtgtttgccccggtgggaagggccgcggcggtggtggggggagcacgaatctctttttctctttcgggtttaaaaaaaaaagcgcaaagttgcatcaggacttcctgacaatctgggagaaggcgggcttcctgcctggagctgtttaatttggagcttcccgagcccaacgaacgtccgtgcccagggcccagccccgctcaccgctgcacccccctctgccggactgaggcggtcccacactttggaaaaaaatagtgtgggttcctccctggtcctcccttgccctactgggctcagtttcgcaggggcgggggccggcctctgccctggtctgggggaggggacacccccggaggctgtggcctggtgtcagggcggggcaggggtccccagtcctggcatctgtgttccctgcttgccgggcagtggtgcccctttcgcgaagcacacccgggtggcttggtgctgcacggcctggcacccctacccttccccgaccctggcctagccgggacccagggtccgcgccctccgcccgggggctccccacgtgtgattgatctgggaagcagtcggatggaattaacccacggacaagtgggacggtttgcattgggagtccgccatggacacggcaggtggggccttttgattgtaaaagccctttcggagcccttgcctcgctccaggtgggagctcgcccagcgctagctttggggatctagagccgcctgcctgaggctcccagacagactgcgttttgatcggtcgcacagaaaggtggtgaaacttggggaagattttctagacaggaatcaatgaaaaccattgaggctggagaggagaggttttgagcaactctcttcagtgcggtcagccctgtgtggactgggcagcctgggacctgctcccagtgcagggtcagatgggccgtaaacagggcccggctgtgttccttcctgtgccttgaaaacaagcaggacagcctggcacagaggcagagtctagagctgacaggccttagagagggaaacaggaaagcttctgaaacgtcccgttcacactgatcgttccatttcctcttgtgtctgagtgggagcgggtgtcctccctgcagggaatgccccccctctcagatggcagctgctccttgggcagagttggcaatgtttttctttaaatgaccagatggtaaatattttcatgtcacaaaatcttcttcttctggtatttttccagccattaaatgtaaaagccctcctgagttcatgggctgtacctaaacaggtgttgagcccgattctgtggcacatgtggtttgctgccccctgggcattggtcagggggcctgggttctgccttctcgattgctatccgcgtgggggatctgggggagggatcactgttcttcttgcttttggcctccttggggaggatggggaggtagcccaggggtgctcacccaggccccgtgtcagtcttctatgaaacttttaaagaatagtgatgactgactgtctgtctgtatggtactttccttaaacctaaaactggtcccaaataaagtctcttaatttgaaagatgctgaagcccgggccataccccacactgattctgtgtctggggatggggcgtggggcctgggcctcactcagtgttttctctcagtcacctgggggagatggaagtggagccggccaagaaccctgcctgcctgcctgctggccgggactcctgagtcaggctctctggccctggggtgtgggcagctccagatggacccgcgatgtgcaggttcagctggcctggccggaggtgggacactggctttgctgtctttggagtgccccctccctctctggcgagctttggctggaagcagttctaccgtgttttggaaatgaatgaggccttcagaaggcattagtcagtgtgtgcctgcgctggctcagacagtgcctggtgagggtttgagtcatcctggggtgcccctggcccccacgccctccctctccagtgcaggatcattacccaaaaatctggcagggagctgccccacccacagggagcaggggcctccttcagcagtctcacctaatgttgctggagccttgggggatcagggcccatctcttctagagagatgtcagggcagggctgggcgcgatggctcacacctgtaatcccagagcttcgggaggccaaggtgggaggattgcttgagcgtagccattcgagagcagcctgggcaacgtagagatccccatctctatgaaaaatatttaaaaattagctgggcatggtggtagtgcacctgtagtcccagctactcaggaggccaaggtgggatgattgtttgagtccaggagttggaggctacagtgagccatgattgtatgactgcactccagcctgggtgacagaccctgtctcaaaaaagaaaaaggaaaaaaaagggcaggacatttgtgattctgataatatgggaccgcacctccagttctatcagtgggaaatctagacagggctgcggaaagccagctggtgcgagaggagccaccgtgtcactgactgtgggacacccacgtgggctgacaatatggcttctgcttttcagggtgcctcgtggcacagcctaggggcacacccacggccggcaagctgggcgtcacctccttcaggctgattgtcactgagaagtgtcaccatttagcatgagggatgctgcctcctttttcagaacattgtcaccatcagggtctcaccactcctgggaggcggccgagaagctggggaacagcaggcactcggctcacagttgctcagcagtgcagaccctctgagctgagcatggcagagtcacccttcggaggcctgtgcccgggtctcaggacctgcacagaaccctggcctgtcccatccgagggtgctgggaagagcatggccgtggcagagtagggtgggagctgctttcctctgtggcttgggggccccttctgagcatcagctccctggtgtgacagaggggcgcactctgtccccatgctgggcctggaggctggatgagtcagcaggagagcctggggcctgcctcacagcaccaagggctgcaggtgtgagtgtgcacatgtgtgcgtgtttggggaaggggccagggactgcccaggagctgaggatgggtcacagcgggtgctcgtcccgcagcgggtcactggtgcccaggacacagggagctccagccccagctgccagggtcccacagagaggaagtttcctctgggggtgggtgggggcgcacagtctctgatcctggccccaaggcagcttcctgggcggtgtctctcctgtgctgactcggcagtgcatttgctttcggtgctcaaagatgaaggggaaccaccgtgggccttgacggcctcatctgcccgctgcagcccactcctgagatgggaccaccgcagtcgtcagggtccagtgagagccgcatcttgcaggaagccattcctggcctctctggcctcagaaatccccttttcaattcaacaaaatgttagtcttctgtttagctattttagaaatagacagttaggcttttttctcttttttcttaaagacagaggctcactctgtcgcccaggctggagtgtagcggcgtgattttggctccctacaacttcagcctccagggctcaagccatcctcctgcctcagcctcctgagtagctgagattacaggtgtgtagcaccatacctaatttttgtattttttgtagagacggggtttcaccactttggccaggctggccttgaactcctgaccttaagcgatctgcccgcctcagcctccaaaagtgctggggttacaggcatgagccaccgcgcccggctgacagttagacttttgcttctttgtttatataagctttttcttctggttccaaaagcaagtttgcccttccttgtggtagagaatcctagctcacagagcagtttagaagccagcacagtatcccacacacacatctggcatggacagacccttccttgctgggtgtgggtcctgtgttcttctgaaaggcaagctgttcccagccaacccctgcccctctctgccttagcctgcctggaggcctgagtctcctgggtgactgtgaggtgggacccccccttcccctacccccacccacatcctctgtatctgccttctgtcctgctcttgacctttgagctcctctgctggcttcagggtgcggctgttgagcctattttttggattaggactctggggtgagggaagttaattcacacacccaagatcacactggtgggaagggacaggcccggggtgaaggcttctcctctccttggcggttgagtcccacacctgctggccgaggcacctgaaggggacttggggtccagggtcactgggaggacgggggcaggcagaggggtggccgacctggtggcggctcgtgggcagcagccgaccctatcttgctctgaacgtgtggggccctcacccccttctctgggtctgggtttcctcccctgtaagtgacaccgtaaaagcttcacagccgcttccaagtctcaggtctctcgggctttggatctcacacccaggctgggtgggggtaggggcgggacagccgtcccccccggaaggctcagaattcctcgcacaatcgtggggccaggagacccgcaacacaggctttcccagctgcgctgagtgccgcggtggccgggggtccgtcgggcctccatggagctgaggggaaggggccactcaccgcctggtcccggagcacacagggcagctcccaggagcacagaggctccttgggacctgtggggctgtcggcctccctcatgctgcacacacagcgcgtccccaggggtgtctgcagcccagcccatcccactgcagattcccgaccactcagattcattcatgcatcctctcacgccggtcctgtgggacagagctctgggcagcagccagaagtccaagttctggttcagggccagtggaggtgggtgttggggtggggctggagctccctgctctccctcccaagctagccaggaaaggaggttgggggccccgcacggtcattgctgtttattcacaaagcgcgatgctgagcacaggcggggaaagaaaagtgcgatcagtgccaggaaaatggggctcccccgacgccgtccaaaatgggatcccttgccgggcgcggtggctcacacctgtaatcccagcactttgggaagccgaggcaggtggatcacctgaggtcaggagttcgagaccagcctgaccaacatggcaaaactccatctcagctaaaaatacaaaaattagctgggcatggtggcgggcacctgtattcccagctgggaaggctgagacaggagaatcgccggaacccaggaggtagaggttgcagtgagccacagtcgtgccactgcactccagcttgggggcttgggggacagcaagactccctctcaaaaaaaaaaaaaaaaagtgaagtcgtaaatcagattaaattccctttttaaccctttgaacctctgtcctcccctgttcccagcgggaagcctctggtgaacgcgccatgcaccccacctgcccccgctctctgggtctctctcccagctggaacggccgcttccccaggtgccttccctgggccacagccttgtgcctcggcggctgctggatgcctgggtgtgtgggtggctcccagtgtgtgggatggcacacgagcctctcgcccttctgtgtggggtcgcacacccaccgcaggccgtatttttgctcacgttcatgtttctccacggtggacgctgggttgcagggacccttcctgtgtgcgggtgaggatctgggcagctgctggtgccgggcccatggggacgctgaccgtcccgggtgccggctctgaggtgtgcagtggacggctgtcctgccgggcgctgccagggccccttaggccgacgtgcgtggccacccgattccccgccgttgtctcaggaacctttgccgagtggggtggatcaatttttcgggtgtgttttaatagcataattacagggagtatttcaggctccctctgacgggccggcagggtttggctgccggctgtttaccaggctccaatctgcacactatttttctgtgggtatatatagctggggctgcttctccttcctcaggttcaggctaaagagggacagcagccgcctcagccaccccctgtggtttcctttgcctgtggatgggcggctaaaatgggcccaggaagagtcaagaacaaggccggctctcggtgccacagctctacccccaaaagcaggaagggggctcgggccatgcccatctgtgagctacaccggtccgggagcggcatcaggcaggggagtcctggacccccgcagtgctggggtgtgtttgtccgccctccctcccgtgtgtctagaagcctccagcctcggggaaaacaatgaaactcaactgtgacttaaacagattcccaggcccgcaggagctcccggaggcttgtggctgtggcgagacctggagggccatgcgggagggacagacgcaggtttgcggaggccgcctgcccaggaggggcgtcaaaggaggggacagatgtgggtttagggaggccacctgcccgggaggagcctcgaaggaaggcacaggcgtgggtttggggctgcctgccctggaggggcctcaaggaccccaggtctggtcttggtctcactcacctcctggaccccccaaggcctgcagtttgcaatctgtcgcctgggacccccactgtctgcctttacgcagctcagccaccacgcggccctcgctccctcatttacttgatttctgtttatggttaaagtaccgtttaaaacgacacatcattaaagcaacatgaaagggagttttgaaaagggaagccatcgtccatcccactgcccctgcctcagcggggatttacttttcctttcctgtctgcgggccagtgacaatgaggaccccgcaatgtgtctgcgggccagtgacaatgaggaccccgcaatgtgtctgcgggccagtgacagtgaggaccccgcaatgtgtctgcgggccagtgacagtgaggaccctgcaatgtgtctgcgggccagtgacaatgaggaccctgcaatgggcggcctgtaaggctctgccctggcctccgctgccttcgctttctccctccttggtgggtgcacgcccttgtgcttttcctaaaagagcaggtcctccgggcatggtggctcacgccggtaatcccagcactttgggaggccgagacgggtggatcccaaggccaggagttcaagaccagcctggccaacatggcaaaaccctgtccctactgaaaatacaaaaattagctgggtatggtgacaggcatctgtaatcctagctactcgggaggctgaggcaggagaatcacttgaatccgggagacggagtttgcagtgagccgagatcacaccattgcactccagcctgggcaacaagagcgaaactccatctcaaaaaagaagaagaagaaaatcctgacacttcagcctggtgcaggcccttccctccttctagtccctgccaagaagtgagccgggcccagatctcctgccgggcggggaatgagcacacacattcccctcttgggacagacagcagcagcagccctgttgcacacatgaggacgtacaggctcaggggccgtgggtggcagagaggctatcagcgccggactggcccgccccgagccagggtccagccccacagtcctgtccccaagccctggcccttctgcggtcactcccgtctgctgaatcccctactctgcccctggtgtgtggccccccagttccctcctgtgttcattccctgctaacctcccgtggcttcgcctccccagatgccctgagcacacagcctctccccttcctcccctcctagatgtgcacataggagccgcccaaaggctggggcagctagtggggcccctccaagggaagctgggccccgggcaatgccctgagccaccaggtcctggccctgcgtctcatcccttcttttttttttttgagacagagtctcgctctgtcgccctggctggagtgcagtggcccagtctgggctcactgcaagctctgcctcccaggttcacgccattctccttcctcagcctcccgagtagctgggactacaggcgcccaccaccacactccgctaattttttgtatttttagtagagacggggtttcaccgtgttaaccaggatggtctcaatctcctgacctcatgatccacccgcctcggcctcccagaatgctgggatgacaggcgtgagccaccgcgcccggcctcatttggttccttctgtgcaccacagtgtgggatctcgggtcctgggtggcacgtgtttaacctgaaaggaaactgcccctgcgctccccagcttgtagcccgtgggcctggctctgaggccccgactgccccacggcctgtgctgcgcatgctggagccaggctccggctctggttggcgcctcccgtggctttaatctgcagtgacctgggtgcttaacgagggcctttgcctctgcgtgtgcactgccttcttctgaggagtctcctcaagtctcccagctgtttaaacaatggggtcttttgtcttttgacctgttggtgccatcagccagcctcctgcacatactctccctacccttggctgccactcctgtcctgcccttcgccatgtcttttttcttttcttttttttttttttttttgacagcgtcttattctgccacccaggctgtagtggagtggcacgatcttggctcactgcaccctccgcctccctggttcaaccgattctcctgccttagcctcccaagtagctaggactacaggtgcccaccaccacacccggctaatttttgtattgttagtggagatggagtttcaccattttggccaggctggtctcaaactcctgaccttaggtgatccgcctgccttggcctcccaaagtgctgggattacaggcgtgagccactgcgccgggcccccgccatgtgtttttaagagcaggcatttcattcagatgaagcccggacactcttgggggttctgctcaggggctctacctgccactgaacgtcctctccctgtgtgggtggccatggcattcagcctgtgttgggccttgttctgcctggctactggccgctaggtctgccccggcatcctctgtgtcctgtgtgggcgcctctgcctcctgctccagcctgtgccaggcaatcctgctcaccttccaggagccaggcctctccccagggcctgcgtcctgtcagggtcagggacggcccctctgccatgctccggagtccctggtcccctcactccgttacgtcctgggtgtcacgggtacggccgggaactctgtcgtcttcactgtctgggccggggcctccctgggtgtctgctggatggagtgggtgcctttgggtccctgcaaagtgagcctgcctcccagcaccgccctgtcgttacatagccactatctttgcgcctgtttttccttcctttgactggttcctctggggttaattcccaggcctggtattaccatctctgaatgcctgggtggtttcagcgcccaggaggctgtgctgaggtatcttagaccatgtgggcaccgttcgctcctgcgcagccggctccggggtgccctgtttttgcggaatcctgcagggaaccccatgtaccctaagagtgctctccccagccactgtggcataagacaagcggtctctttgcccttgggccccatccttgtctggtcggcccttcttcatgggtccagcgcgggattgccggcttccttttcaggcttcctgggacccccactcagacctgcagctgggccagcgatgcccacccgtttctcctccacgtggtatacagaggtgcccaggctgctgctggggactctggagcccaggagtgagtctccttgaccctgagctgtcctggctatcacagctgggtcctgttttccccttcagcacccacgggtgtctttctccagtttatattgttatttttatttatttacttatcgagacagagtctcgctctgtcgcccaagctggtgtgcagtggcacaatctcgactcatcgcaaactccgcctcccgggttcaagcgattctcatgcctcagcctcctgagtagctgggattacaggcatgtatcaccaggctggacctctagtttatattattacagcctggtcagggagtcactgggcgtcgccatcctgtgggtgggaagggggcccaggcagaggccaggaggaggtgacagtcatgcgcttagaagctcaggccacgcccacccagccctgcctggtgaccggttcctgctgtgttgggagctgcatcccagaccttatcgccgggcacagaacttccaagccaggggagagggaggcctggaggggccccaatctctgaaggtcagcagtggcggggaggaggcttgcggtgctgaagggactcgggggacctgcagggaggtgttggtggtcagggatggtggcacctgaggggacttttggcagggccagaagtgcccagagcaagctccggtggggccctgcactggagggctggggtcgagtgaccctcttcctaagaccacccaggaggacactgggtgcagggtggccggagccctcacccccagtaggcagctgctgtccactccgccgacctgcctgtcacccagtaggcagctgctgtccactcccccgacctgcctgtcacccagtaggcagctgctgtccactcccccgacctgcctgtcacccaataggcagctgctgtccagtcccccgacctgcctgtcagccttttccctgtcaggccctgttcctaggagcctggagacctcaggggtggccttgagcccccagggtttttttgaggggaagcgccagctgctgtcttcacccttcccctagtgaggccaggctgtgcagggccacgtggaggcagtctgtgctgcgcccatcggtcgcctggcttcctgccgaccctcggcccccagccacctctggtctcgggcaaggcccctccccctgcccacctcctccctggcccccacgccaggtgggcagacctcctctgcggtttttattcagggggtccctcgttggctgcccactcttggagggctgtcctgactcaggcctcccctctactcagatcccctgagcgagggcctgggcgtgacgccgggagttactggggggccagagggggaggctcagcctgaatcaatgagacccaggaggaaggaggcacgtggacctgagggctggctggagccgctggtgacagatggaggagtaattgctgcttccagagcacagcgagctcgagctccctggagtgccagaagcttctgggtggacagacaggccgcctcacattccagaggctgacacagtcttccaggcacccctggggccagctggaagccatgtgcctccactcacgtgtcccgtgggtgtttggaggggaggctggccctgccatggcccaccccagcctgcggcctcaggagcttgcacatttgcaagggggtgacatgaagactgagccagggctgcggcgggcatccccctcagagaacagggaggagggggcacaggcctttttttttttttttttgacagagtctcactctttggccaggctggaatgcagtggcacgatctcagctcactgccaccttcgcctcccaggttcaagcgattctcctgcctcagcctccccagtagctgagattacaggcacccaccatcacgcccggctcatttttgtatttttagtagagacggggttttaccatgttgtccaggatggtcttgatctgttgacctcgtgatctgcttgcctcggcctcccaaagtgctgggattacaggcgtgagccactgtgccctgccaggcacgggcctttttatgagggaggaagccgtgccctctgccacctgcctgtgggctggggcctgcaggctcccagggccctcagctccagcgtggctgttggttattggcacctgggcctcatgtccacatggaaagtatattccgagctggtggctaagccacaagagcctgcttacctgtcccaacccccggctcacttgctgccatgatacgtctgggattctgggccctccttctgagcttggacacagacttgggacttcagcgctggacacaggtgctggatctggggtctcaatggcaccagggatggtcattctgacagccatgcccagagtctcaggagggcctggggccgcaggtggacaggcatcctgaccagagtctcaggagggcctggggccgcgggtggacaggcatagagtctcaggtgggcctggggccgcgggtggacgggcatagagtctcaggagggcctggggccgcgggtggatgggcatagagtctcaggagggcctggggccgcgggtggacgggcatagagtctcaggtgggcctggggccgcgggtggacgggcatagagtctcaggagggcctggggccgcgggtggacgggcatagagtctcaggagggcctggggccgcgggtggacgggcatagagtctcaggagggcctggggccgcgggtggacgggcatagagtctcaggagggcctggggccgcgggtggacgggcatagagtctcaggagggcctggggccgcgggtggacgggcatctggacgtcggctccactagtgtcacctctgcaaccttgtcccacccagcacctccctatggccctgctctgactgtgggctgagggggacccccatggctagcttgggacctccgctggacactgtcatagggcacttgtcgagtggccctgctgaggttcaggcttgggcgtgtgtggcccctgagcccagcagctgcgtgagccgtggggagccgagcccccagtcaagaaagctgtgtgctccttaccctgcctgctgggcttggggcctgcagggcaagggaggcggtgggatgggagccccgcctggcctggtttcttgttgtcgccgcactcctagctgtatgtagtcagatgaggctcccagtcctggctctgctgctgagcaccattgggccggtggttgggtgaatctctcagcctctctgagcctccagcacttcgtccttaagagtggaactggtctggacctcccaagggggggtcactgggtgcagagttcctgcaaggctgggcccggtgccagtagcggtcgctctgtggggcctttcgcacggttgatttttatctccctgtgagattagcgcctgccctgctctgcctcacggctctggctctccgggactgagaccacctgctaagtgacaggggcggaaggaccttgcaacacagagcaagacgtgatagggtggagctgctccgcccaggccccgcctgcagatgagagggcccagagcctcttaatcccctgcgctcagggcatgtgacggcagggagtctctccagtgccgcccaccggattcctatagttagagctcctcgcccaagcccccagggcacctcactggcctcccaggtgaggacatgaggcccagcgactctggtggtggctggtgtcacctatggcagggccgcgcggggcccagtggaggacgcctggcccggacctgactgctccgtgggaaccgtggggcgtgctcagggtgacttggtgcggctgggctgccagccggcctggctgagtcactggcagtgaaggcaccaggtggtggacgtgctcggcagctggcgggagagtacccccacccaggaccgtgttcaggctgagggggaagggagcggcccaggcaggcaccgcccatggcggggcccccgcactaacggccacctctcccgatggactgcagttctggagccgcccctgaggagaacgccctgctcagtgtcctggcagactctggactcttcaccgtgccatcctcgctacagcctggccaggcagccgctcccgtccccccaccccacagacaggaactgcagactcctaaaggtcgagccagctcccaagtccatagccagaaagtgatgcaggcggggcccggctggggggcaggtgtgaccgggtcatgggggagcgggctgtgcacaggcatcaggctgagaggtctcggggatacgtcctgggagccgcctgccaggcgtcctgtggggctgcctgcaggcctcctctggctttggcaggttctgtcccgacagaccgaggcttgggaagaccggattgtgcactctctgcctggagagagggtggggaggggctggggcgtgtgggcagggagaacaccctgggaggcatcagtcctcttccctggggacgggccatgcgtcaacagtccctcacttcctctctcaggggcagaggcgtgggggtcccgagcctccaggttggagtaggttaggagggcctcagagccccctgctgccccgccatgtggcattggaaggggtgtgaccccctaggggatctgttaaccacactccgccccatgccggcctctctgttccctctaacctgcgcaggagcagggccagctctgagctagcagaggtgacatgaggctcgtcctggccccgcccaccctggcccctccctgtttcccaccacgctccgcccaccagagctacatgttgtgtttgagcctcagccccagacctggctcaggtcctcaggaggaagcagtgacagccaggcccggggtcctctccctgctctgctccctgcgtgctgactggaggctgcaggtccccaggcttggccctgaccctcaggaatggagccggccgatgtgaggtgggggctccggtcatgtgcagtggtaggagaggaggcgggaccggtcccacagctccattgctgccgaggcgttccgcaggtctgtcttcatattggtaaggaaaatgcgaggatggtgtagcctgggcatcccagtccccaagtccgaaatctaaatccaagcggaaaattccaggcctgacttcatacgccaggtcacagtcagaagccagaattattgaaagtatgctctgggcgtggtggcctcacacctgtaatcccagcactttgggaggccatggtgggaggatcacttgaggccaggagtttgagagcagcctgggtaacatagtgagacccccgtcattatttacacaaaattatgtgactgcctttagggtatgtgtacgaggtatatattgaaatgtgagtagaattttgtgttgagtcccatccccaagatacctcattatgcgtgtgcaaatattccaaaatccagaaaatcctaaactggaaatacttctggcccctttggatgaggggcccccactctgcatagcaagtgtgggcgcgggtgctgctgtgtcctagcgtacttcagtgtgtggcctttgcagtgaatagggctggtgtcctcactgtacagatgaggaaactgaggcccagcttgctttgccaaggtgcatccggccccggccatggctattctggctccagatcccatggtctgcagccacaatactgctgtgccccggactgggccctgcagctcgcggtgtcgctggcctgcccattgtgggcaccgcccccaccccagactggccgaggcctagaagggagcagggcctggctgaggctgcaggggtggggacggtcagccagcccctcactgccaggaagggcgcatccatcctggcctctccccagggagaagggaggagcggctgagagggaagcgctcttgccctgtggacgagctcctgccccacggactagggagcccccgcccacaacctgcttgtcagggccacccgggacccccgggagttcggctgctcgctctgctgttaggaattggattagttttccataaaaacaggatgtggtgggtgagagggcagtgtgtccgtctttctcactcccctttttccaggaactgagcacgcgcataggttttagccagggccgtccagtcccctccccaccccccacagggaacaatccactctctgctcttaagtggccacttaatcagcttctcctcctggcccggggagcttcttggagccggcctgccgtggtgggaacagctatggggacaccctgccataaggtccagcagctaagctgggatgtggggggaggggctgcgaggcccaggcagtgtgccaggccgcacaagaggagcccagctcttgccccaccagctggcagccctggaccgaggttgggcccgtgaggttggctgggccctgggccctgggcccccctccccaggacacgactgtggtggcacatggctttgggggctcgtgggtcccactttgcagacctctgctttaaggggtctggtccacggggtcccctctggagggcctgggggaaatctcagggacctggggtctggacccgggggagggagcgggagaagcatgtgcgtgagtctcgtgctgtcagggagcccgggaagtctgcgagggcttgggggttgtgtcagggagtgtgggttttgcccttcagtggtggaagctggcttgagtcccctcgatccctcaaggctgtagtcctgactcggggctgtagggcagggcagggtggggtcaccctgaggcagaaggctcagcggagatgttctggcttggctctgcccctccctggctgggtggcctcaccctgtgacctttggggaccctggttcctctgagccaggggacagcagtgactccgccttcctaggtggctgaggatgacatgggctccccctgcaaatgtgggttctggctcagtggccaagtgtatgatggtatgtggctcttggggtcctgagagagatgggagaggagcaggggtttgtagggaagctggcggcttccaccccagccagtcacctgcagtgggggagttccaaagctgactgaagcttcgaccttgtggctggtccccttccttcctgcctcagtcattctggtctctgggggatcagggctggggggctctgggctgtgggggcctgtttttgtgacttaaagctctcccagcacagccccctgacctccttcctcatgggcaggacctggcccaggggtctcagcacagccacaggccagggatgcccttgcagatggccctggatggaattccagaactcagaaatgtctccttcccgtaaggatgtcccgagactcatgagaccgtttccttctgggaagggggaggaatggggagatgagtgaagagcgcactgcagctcaatccgggaagaagctaatcaatcaatcagggaagccaatcgatcggagaagctgatgggaaagctgtgcttggtagaataggctcgtgcgggcagagcagtcgcggcactcacaggctgactgtgaggaccttgggtgttactttgtgcttctctgcattttaaaaacttttgaaagtggagaagaggaaagtgaatgttctctgagatttcatggaaaggggaaactgaggcccactctagccagtttgggcccagggttccaacctggggtggccccggccctcgtggcctgaggtgatcgtccctgtggctctgagagcagctggggccgggtccccgttctggggctggtgatcctggggaagagccaggcagtgccctgcccacctagtggttatgagcccagaatgttgatttttttcccttggttgcttcatgactttgttgaatttccagagtatgtgtgggggcccccggcgtcccactcgccccagccctgtggcagcagagctggctgtcaagctcagtcagctgggcccagggccccggaggtaggtgggtgtgtgcctgagcttcccctttgggccctgccaggtgctgggagggaccacacaggcggcaggaactcggggtccccaggcctcggccacaccagcctggtgcttgttatatattgatatgtctctctacctgtgaaatgggtatttattttaaggagctgacgcacgcgattgtggggctgtcacgtctgaagttcgcagggcgcgctggctgtcaagagccgctgttgcagtctcgagtccaggctgtgcgctcaggccgggcttctctgtggcggtcctgggaattcctcctccgggcccttaggcgacactcccctgccttcagctgattggatgaggccctcatgccgtctgctgatttaaatcaatctcattttaaaaacacctgcacaccaaattgcgattggcgtttgactaaactgggcagcgtggcccagcagcgctgacacatgaatcaaccctcacaccccacccgcaggcgtgaccacggcacccacgctgccgactgagaacacagccgtgcgctgactcgcatgtgatgtctctggtcgcacctcctccatcctcagcaccctgttcagaatggagatagcggccgggtgcagtgctcacacctgtatccccagcaccttgggaggcctgggtgggcgggtcacctgaggtcaggagttcgagaccagcctggccaacatggtgaaaccccatctctactgaaaatagaaaaattagccgggtgtggtggcaggtgtctgtagtcccagctactcgggaggctgaggcaggagaatcgcttgaacccaggaggtagaggttgtagtgcgcgagattgtgccactgcactccagcctgggcgggcgacagagtgagactctgtctcaaaaaaaaaaaaaaaaaaaattagagataacgacttgggctctctagagaccagggagccaggctccaggcgctgctgtccagccccttgccagctatacgaggtgctcacctggccacgtgtccgggcagtgcttctggggtggcatccactgggagggcaagatggttctggtacaggtgcccaattctgtccccatttcacttactgggaactcaaggcacagagaggggagggctgagctaggaccagaccccagtctcctgcagaagtacacagacatgatgtacgaccatcctggacacctgccctgagattcccctccctctcctgccctgtcccagtggcctggggggaaggggaagcaaggttctgaagggagtgtgaccagacacctgcccgtgacaccccctctccaggctgcctccgagtggctggtgactcccctcctgcctgcgagggaggtggccaggttgcattcctctctgagtgccggggaagtccctagagagcaggccagcctgtgactgggccctggggcagtctagacaggccagactggacaggccagggggctgggtgccgctgggtaaatcacagggtgagggctctgagtcagcaccccatcttctgtcctgggtccagcaccgctgaggacacagtgggcagccgggtctgccagggccaggtagctgtgttgagaaggcagtgctcctgagaggcggctaccgggaggttttcaatggccaggcttcttaggaagcccttgttgcctctctggggtgagttgctggggccatggttggagtggtcgccagtgtctgcccctggtgccgagggcggagtcctcgttttgggaggtcacggcatgatgctgggagtcaaaggcaggccgtggcaggggcattccttttttctttcttttttttttttttttgagacggagtttcactcttgtcgcccaggctggagtgcagtggtgcgatcccagctcactgggatcccaggctcccaggttcaagcgattctcctgcctcagcctcccgagtagctgggattacaggtacgtgccaccatgcccggctaatttttgtatttttagtagcgacggggtttcgtcatgttggccaggctggtctcgaactcctgacctcatgatccacccgccttagcttcccaaagtgttggcattacaggtgtgagccaccgcgcccggcctggcaggggaatgtcgacgcgtgatctctgcctggagagcacgttcatgtttcccagaggacactttagaacatggcgcctgggtttggatgaacctcagcctaagaatctacctgctcaggatccagcgacgctggtggtgtggacttcagctctggagaatgggttatatggaacctgggcgccgggagggcattgccacgtgcttgctgctggggcttcaagaggaccccatctcctgtggccgagaccccgtgtctcaaggcacatcccctttcgtaccccgccccaccctccgcagcttcatgacctctgggtttcccccaggaccttcgcatctgatgttcccagatccttcctgccactgggtcctgctctggtgccccccggggaagccttccctgaggacccagctcagcatctggtgctaactgtggctcatcgtgcactttggcccccaggaggctgtgggctcctgaaacccctctgaaccacgggcttccaaccacacctgaccccctgcgtgccgaccctgtgtgcaggtgtacaggtgtgcctggggcaggatggctgtgacggcctcacagagcccggagagctgcctcctagcttccaaagccttcatttcaggaatcttaccctctcaattagtctggaatgctgggggcggggccagctccaggtcacagagcgaccttgtttacccagaccttaacatcggcccttccatgctaatcaatgtaatcattgtggtccatgcggcctctggaatgtgctgtccactccctgggtcagccagagagtgtcagggagcacctaccggctgttacccagtgctgccctgacctggttcttcactctgcacatttgtatcacgccagaccctggctggcagctccaggtgacgaggcatgtcagtgccttcctgttctgttctgttttgttttgttttttaaatcgggatgaggccttcctgtgttgcccaggttggtcttgaactctcagggtcaagcgaaccttctgccttggcctcataaactgctggattacaggcaggagtcaccatacctggcccactgctactttctagatgaagagacagaatcccagagaagaagcaggggtttggctgctggtctggagccggttctgctcacctccagcttctgccttgggccgccctgttcacacaggagctgctcacaggctgagacctcgagcagggccctcctagaggaactgggcccccgtaagtgccctgagccgccaggagccggccctgcgtctcatccctatctccggaggacattggctgctagctcaccagctggcccctgggcaggcttgaatcatgacctggaacgccaggtgtctctggctctacccctggacctgcaccctgtccaagtgccccagggccagactgttttggttgcaccctctggacgggctacccccatgatggctgctcatggaaagctgtggttcttagggagctgccaattcctagtcctgcagcctggagctcctgggtataaggtgggggctcgggcgtattggggactgggggtctcaggaaagagcctgtgggacctgtgaactcatagctgctggccgagggaccaccttgtggctgtccttctcagctaggcctggtcagggcttgtgtgcagggcggctgaagctgtgggaggccacactgtccacacagtgccctgtaagcccaccgtgcctcagtttccccgtctgacaagtggcacaacagaagccacttcctggcacacagctcagggtcagggccgacacagcacttgtgggctgccgggagacccgagaggctgccccttccttgccttggctgccacgggtgacctggcaaacccctctggccgtggcaccactgggggtctacccttggcagtcagggttggccgcttggctgggagccccttctcctccccagacacatcctctccttggggctggagggggtcctgccgtccccgggattgtcgagcagcaggaatccaggagggcagtgcctgcagctcagatgggggccagtgggcagggccgatccaagggtggcaggaaagtgcccatcactgacctcaggtgggggaggccatggtgtgtgaaggaaggagagctgagtgggaggtcttactttgtcaccgcccctctgagtgcctgctgtgtgcaaaggccagcgggggccctttcttcagctgggctctgcccagacccctgagctctgggtgggccgggagggagaccttgctgctcacagaggtggctctgcctgacccagctcccttcccagggcacagtgggggcatagggtcggctccgtcagacattccgggacctgcgtccttcctggggccacaccctctacccactgtcccccacctatttacctgtatctgcgccagagatggctgcccagataagccctggtttcctccctttctggagaggctgcgggggctggcgaggaacccacctgcgcagagagtcaggggattgctctgtgtggaacgcaggcctcacccatgccctggaatctgtccccttctctgttgctgagggatgagtcccagatccctgaccctgcaggggagcccagcacagaaaaactctgaggcctccacaccctggcagcgctgctggtcgtctgtggggaaggacaggccctgggagggagggggaggtgcggagggcagtggggagggtcaggaggaagtgggggaagggccacccaggccccgatgtgggggatgtctcacgcgtggggtggggcattctcatctctgcttggtctcctgccatgctgggggtcgttcactgcggaccccaagtaccatgaagatggggatgggatgctgagcagcatcggggagaacgcaaaggcacctcccagctcacccgcccccaccccgcaagcacaaccattgccatggtgtggggaccggaaggcggcggctttgggaccagactgcttctgcctcgggccgtgccgctgggcctttggtcagcaccatcgtgccctgcaagtcactcttagcctggtgccctcctgggcagggcagtgccacaagagctcaggcccagatgtgcaggtgccactgttccacccaccagcaggtcacctggggaaccctcccctcctgcagcctctgtgtgctcatctgtgaaatgggcgtggtggagtcacccctggcttgtgggagaatcccaggggctgatgcctgcaggaccctgtgggctttgccccgctccctgggcagagacagttcccccagtcccacccacgtggctgtgtgcagcaggtgcctgctgaccctctgttcctgcacagtcaccttcttcacagacggacccccaccctgccctgcaaacccctccaggggctgcgggctgagtgtgtccgggagggtgtcctgactctccacgccagcaggtctgagagcagatggctgtggcaggtgcggtgggtgcccagcccacagcagccaccaggcctgcaggaccctgccccgtgtaggtcagatgagccataaaactgagtttcctggacactgagctaattaaacctggacaccgagctaattaaatggtccagaagctcctcagtgccccaggctgctggccgggctccaagtaggtgaggaacattccgtttacctcctgctgcgtcgaaggcgggtggctcccctcgggcccctgcctgtcccgggccccctgggtgctgctgcgtcaaaggcgggtgtctccgcttgggaccctgcctgtcctgggcttcctgggtgctgctgcctcgaagacgggtggctcccctcgggcccctgcctgtcctgggctccctgggtcctgctgccttaaaggcgggtcgttcccctcggatccctgcctgtcttgagctccctgggtgctgcctgccctgtggccacgtcccactgttgcctttggacaaagctctcctagggcctggggttctcccatgagatgacaggggttggttcaaaggtctctgaggtttttagagctttgtgaagtgttctagaatccattttctctctcattgctggacagagagtatagactgggctttttcttgagtttctctcaactcttctttgtccatgaggcaggaagaggggcttcctcagtcctcagcttggggtggattgggatggacagagaaccgtgcaggatcccagcctgagacggtccagcgccccgggggagcggagcccgtggctcagccgtctgtagccacggccggggtcactgtcactgagggcacggaggccccgccggcgaggtccgaggtgggcgtgtggggtggtgggcgctggaggcaggacctctgcttgtggagggtgggccaggcgtggaccaggtgtcacgtccgctggggcctttgaggggcaggtggggattggcgcggagaaggagtgaagcagctggggttttgggagcctgtgcggagcaggcccggatgccagggtggctggtgaaggtgggcctggccgggctcggcctccattgggggagccccccaggtcccctccccacacagcttccccctctgtctgctgtccaaggctcctgtgctggcactctggggtggtaggccatgcagcccgtgtgaacctccatagaccttgctgtgaacgctgcacggggcgtctgggggcgggctggcttccccccgtcccctgggccaaccttgccagccttcttcttccataaaagtgggatccgtctgagccctcatggcccctctgggtctgggtttgctttttgtgctctgcctggggtcatggcagggaaggcccagcaggctcccttgcagagcagggcagagcagcggccgccaggagctgcctgtaccacgtctgctcttcttcctctcttcctctgcccggccccgcccaccgtcgaaagcactagcacgggagtgtttatcggtttctcttccaagccaaataaggcagagagcgctcttgcaggagttggagcaggccagggggagggcagctggggcttggaccaggaccccggctccctgtagctgccctggcctggcagctgtcatccgcgaactctgatcctcgcctgccctcacccggcccctttcagagcttcccatgctcagctggtagcaaaagaagtcaagacctagcaaggtgcctgccccggccaggaggcccaggttctagccctgcagctgccgctgtgagctctggggactcagacgactgatgtccttcccagcttctgtttcctttgatgagaggaaggttggaccaagcgacctgccctgcttctgtctgtttcctccagtccttttcctttttgaccagttcacttgttgataactccagcaacgcatgaaaacattccccttgtaaaaaagggaaatgccgtgggtaggggggaccaaggacctcttctgcaggagcagacgcaacagcttggtgtggatcttcctcagcctttttgtccatcctagacatgtggaatttcagttttacacaaaaggaatggtaggcgtctgactctctgtggcttgtatcacttggcagtgccacagggattggtgcatgtttgctctctcatgctatgtgtcaggcactgttgtctctgcgacaatcctgtgaggagggagttatggttcttgatttatagacgaacaaactaagacagaggagattgggctcatctgtggtcatctcagcagttgtgagaggtcagggccagagcccagtggtgtcattctgcagggcacatacagacacgacccacagggttctgccgcaccccctgccgcttggcctgctctgcaggtgggtgccgaggctgttcctgcatctgctgtgtcttgtgagtccgtgggtgcctgtggagtgggggcagtgggtttgcatttccaagcactgcctctgtcataggctcagggagaagcagttacgcatgagctgctatgagccacgggtatgactggcatcacagcaggaggagccctggggatggctgagtgacgatgggtggggacagagctcacagaagccagggttgcccccaggccaggccactgctggggccaaggctgggatgcagcacgatgttggtctgtcagggagtggcaggaagcccacagggtcagctgacacttaacccagagtggtgggagccttgaatgccagactgagggccacacagttggtctcggtgcacaaggacttgggctgagagggctgttgctcctcaatggccatctccttgtgggaggagagtccgggcagccgcttccaggaacccacccatgcttgaaatagtgggaccacagggctgaggaggctcctggggattcctcccaggattcagctgctctgtccccaaccccggagggcctattcgtctagccctatatcctctctgccagttaggtcagggcagagaagtagaggcacagagggtggcggaggggtgtccagccaggcctttctgtggcaccttctgaggctggctggagtctgtgaaatctgtgataactggcccagacccttcctgcctcctggggcatctgctggagctgaggctgctgggggagtctgcctgtgacttgagtctcttgctgggccatgctgggctcagttcgcctgtctgtggggtgggatggtgccacccttaggttgttgggaggacccaaggagagtgatgcctccagccatggcagctggcccagctccggcccgcagcctggctccttcagggccaggaacccccaggtcatggactccaaccctcgggctctcctgcttcccaggtgacgaagcttcaacccatgggctctccttcctgggtgtggaagccctggagaaggtggagatgggatctcagtccagcccattggctccacttcctttgagaagctctttcccccgtcttggcccccagcccttgttcaagcacctgtccctctcctgtctcctaggccccgtcagtccttttggagacctgttcccacccgcccctgctctcacaggctgccagtgtccacacactctcaggcactgtcattggagccttttaaccacacgggaaagcaggcaggttaggtaactaccccccacccccccgccagcaacgccccctgcatacccagggcctgcaccaggtgctgctgcgctgccagctctctcgaggtccctcctcctaacctcaatgcatcgcgtcttccagcccccggctccgagggctcagcctccaggtggtctaacctggagtctaaacctggattgccatctgcctgcctcagcccttcccttccccagggaccgagggccagtgcggctccccagccacccattttttgtttgttttgagacggagtctcgctctgtcgcccaggctggagtgcagtgtcctgatctcggctcactgcaagctccatctcctgggttcacgccattctcctgcctcagccccccaagtagctgggactacaggtgcccgccaccacacccggctacttttttgtatttttagtagagacagggtttcaccatgttggccaggatggtctcgatctcctgaccttctgatctgcccgcctcggcctcccaaagtgctgggattacaggcatgagccactgcacctggcttgtttgtttttatttttattgttttttgagacggaatcttgctctattgcccaggctggagtgcagtgacataatctcagctcactgcaacctccacctcccaggttcaagcgattctcttgcctcagcctcccaagtagctgggactacaggcacccaccaccacacccagatacattttgtatttttagtagagatggggtttcaccatgttggccaggctggtttcgaactcctgaccatgagatggcgggcttgagccatcttcccgcctcggcctcccaaagtgctgggattacaggcgtgagccacggtgcccggccccagccaccagttttgtacagcactcaggtgggtgtggttcctgaggacatgtcacacgagatccttccggtccattagcccaccccgccccatcagtggccagtgcggccattgtggggtccagagtcccgaggcagaacgactgactccaggttgtggaggggcctcttaggatccttctaggcacccaggttgggcaggtgcctccatgcctaagactgagctcctggtggacatcgggctgggtgtgggcgtcctgcacaccctccctgtggcctggtgcccgtgaggagtggacagtcaccccgagagcatagaccaccctcgaggctcccagatggcggccgcagagccccacttccctgcctggtgtgtgataccttccatggctgaggacacctctgactgctcactcctgtgaccctggacccaagtgctgggccacacctggactccaggccccagtccttccttcttctgctgtcctggctcctgggtggcccccgccctccccgctccgaggctctgccctgtgctgggaacccaggaattgccaccccctggccccggtttctcatgtcaggatctgctggccaggttgactcctgagcgccactgtctcctcagacttgctggtcccacccggtccccacctgtccaccgcccgaggctctcctgtgaggccgctctgcagctcttggcctgggggcccccggcctctcatggtgccttctgcactgtcccctttggagatgggagctttgagggtaggcgccaccgttcggtgaaaaggcggtataagcaaagcaacccccagatactgaaggagccgggaaataaaaggaggcagacagagcaagtgtgttggtacccgcctatttactggcaggaacttacagacggaaacatggcctcaggcagcctccaggcaggtagagctctgaacccaaacgcccgatctggggctcgtatcgtgccctgggaggaatgtgcaggtggctgggaacgtggcgggtggggtggccagattcctgctgcagcaccgggtttgtttaggaagaaacgtacgaggactagacactcttttttttctttcctgcacgtgaatgccagggagtaggtgctcctgcaggaagatgatgcatcaaccagccagtctggaggcattccgagacccggggttaatcagcagattagcatttaaataaagttactctgtccccacagccagctaggcccgagccacatggcgggggcggcgggggcggctgttcgccgcatcccaggcttgctccatctcctcgtctgcaatgtggaggtgacagtcgtggtcctcggctagtgccacaggactgtacgggacagatcacccagccccgtgcctgcactgggggcggcggtgacgtgatggccgcggcggtgacctgatggccgcaggtgtgtccaccctctggttaggcctctcctctccctggggcgcaacaggtgtcctcgggtgggaggttcagctgctgggcctggggccccagctttcagctcctgtgcaggcgtggagcgggacggcacgccggggcgttcgttcacacgatgcccccagctcgtctctgcctgctctgtgatgcagcctcagctcctgtgggtcccgggtcacccacccgtgtgggccgcagtctttctgcaccacgtcctgctctcggccagcgctggcctgcgggccccggcagtgtggggtcacacacaggccgcaccggctgtttcacggagcccccctgctcaaaatcctggccttgggtctctgtgtggctcctggagggagcatgtatgaggtgtccaggttgtgaaagccccatccggcagccctccctgtgacagtccttcaggcctcgtcaggcttggttcagcccgtgttagaggaggccagacagctcctcctcgatcaccacagggaacgagggttgggcagtttctcctctcccacccgggcgtgggtcagctgcaagggtctcatcccaggaactggatcctggcaggggggctcaggcatctgacatcccctggcaggtcttcctatgtgccagtgggagtgggtggtgtccagccctctttgtggaatgttccggttgagtggtgtgtggtcctggttaccaccatgtggcatttgtggctttcctggccagcacccactgaaagcagaggccagcccagcccttggacacccaggggcccagcagctaccgtgggggcagcctctcccctcctgactgtgctcctctcagctgtaggatgaaggtctgtggatgggtgatggctgggctctctgcttcccaaggagctggatgtgggccatagtcaggcgtgtgctggtgaggcgagggggttgggggttgggaaccacagctctctctgaccccatcccattgcagctgactcaggaaaaggcattacccccacggggtcacaggcccagcctgggcagctcctgatgggaacatgggagccacagggcagggcaggctcctgtccccgctccttggattgtctcaggccccgcctcccctttggctgaatttcttccttctctgcctgagcctgatctgcgaagcttccgacctgccctgagttggagccagtcttcagggccaaaagcaatgccgtctcctccaggcagcctgctctgaagtctccccctctggctttagcccacaaagtcacagctgaggccacatcaacacacttagaccaagagcactgccggctgcatagacagcacaggtagatccaaggagtgtttcgaaaagccgtggccctgcggccgggatgcccggacctgggtcctgaccactcttgggagctcctcccctctcagagcccatcccatctgaaaatgggggcattggagcattggaggagtgctcctcactcctgccctgctagccggctactccgaggaccccaagaccagatgatgggagaagtggtgggctgggctgtgaccctgagcccccttctcatcccacccgtgaggctgcccctgcttggtgtctgtggcaaggctgacagaagatggcgccagggaccagccagggccctcctgtctcagcccgtccttgggtgagtgggtgtgctctgggggtggcaggtgtgctccgggggcgggaggtgtgctgcggggggccgggtacgctctgggggggcgggtgagctctggggggctgggtgcgctctgggggggctggtgtgctctggggatggacaggtgtgctctggggggcggggtgtgctctggggatggataggtgtgctctgggggggcggttgtgctctgggggggcaggggtgctccgggggtgagtgtgctctggggggcggtgggtgtgctctgggggcggtgggtgggctttgggctaagtagccctcttcctctctgagccttttccttgtctgtgttgttggtgagtggccgccacctgggacaagccttagctgtctgtccaactgtccaccatgtccccggaccctagaccaagcccgctgcctggtggggcctgcttggtattgaatgaatgaatgaatggatgaatggatgaatggatgaatgaatgagtgaacaaactctggggggcgtgttgctgatcaccccagggcaggcccgtggtgggtcatggtctcaggcaggggacttgccctgccgggtgacgttggcctgccggggaacccctgccaaggtgcctcccatgcccccatcgtcctctgcctttgagtccactctgcccctcaaggttcccctctggctcggccaggggcagggcggtcagggaggcctccagctccagcccctccctcatctccatcctcagcccctgcacccgcctcatctccagccccagccccttgcagcctcaggctcgggcttctgagaatcctttgcagatttcagggctggttatttttttattctggcaaaatatacatccataaagctttgtttcctgagatgatctcaccctgtcgcccaggctggagtgcggcagcgtgatcatggctcactgcggcctcagcctcctgggctcaagtgatcctcctgctccagcctcctgagtagctgggaccacaggcatgcaccatcatccccggctaatttttgaatttttttgtagagatggggtctctgtgttgcctggtctggtctcgaactcctgggctcaagtgatccgcctgccttggcctcccaaagtgctgggattacaggcctcagccaccacacccggcctaaagtttgtcacgttagccgcattgaagggcacaggtcagcagcggtaagcatgttcgcattgttgtgcagccatcactgacacccatctctagaacttcttcgttttcccaaaggaaactgcacgcacggcaccacctccctggcctccccacagcctcagggtctggtgaccttcatccccaggacctacgcttctgactccaggagccctgcctggtgtccacaccacactaaggtgccctgccacgggcttcgaacccaaccctggtgcacttgttgagcattggacgttcctggcaggtcagaccgtgagctcctctgctctgacggatgcatggacggctgccacctggctggacaggtgcagaggggaggtgccaccttctctggggacaggactggggcagaactcacccggctgaaaagtgcagctgtggagaacttcagaacttcagaagcctttgctgtgaatgcattttcctcctgcctcttgggccagatcttagggattttttttttttttaatgaaaatgtataatcgtcaaaaaactttagatttaaaagcatggagccgatggctatgcttggtgcgttaatgggaggaagaggggatcttaacttcagggagggctcctgggggagctgggggaggctgctgtgtccagcagggcgggcggtgccccccggagcccggcactccgcgatgtgtgcgctaagccgaggccgccttgagcccgtagcagcgccgagcgcgattctttcgtgtctgcttccgggagggtggaagggtgaagctgttgagagtgggaagggaggggctgtgcttcttgagtttgccgtgtgcccctgaccctttcaggtgcaagcgtcagctccacggtgccaatggggagatgggtctggaggccccaccaggctgtgaaaggcccggcctcctgtgctgtccgtggaggtcggggtctccctctgccctgcgcctcctctaacttgccctgcgttttccgtgcccctggtctagggtgaggctcgggtcttggggactgaggggcaggtgggtgtcaaggtgagagctgggctgggctgggcctccctccagaagacttcccggggctcctttggcaccaaggatggggcagatggtggcacgcatggcctcccctgggcacagagccagactatggagggatctcgttggctacatcctggctggggctttggggtcatggtgggagcagcagccaggggtctcgcttggacacgggtctgagctcactgtggcctccttcctcagcctcctgaccggggtcctgaggctggagggtgggtggagggtggagggtgggtggatagtgggctggaggatgggctgctggcgccccttaggcagcatgaggcgcctttccagtcccagtgtcctccctggtagccccggaaaggctgagtggtccctcaggtcccctgcgaggagacgacatcaggccccacccctcatctcctgacaaacctcacattcctaggaggaagcaggcctggctagcacgtggcaggcacagcctccctgactccagaccttatcagatcagtgcaagtgccagggagaccccgggtgggagctgtgtggttgggactgatgcaggcactggccggactctcaggatgagggtgggaggccaggccccgggaccttctgggacaggcaggagggcagacacgggacatggtgtgggggctgtggcgagtgcggccacgcagagcatttgggctgaaggcgcgctgtgtcccactgccccatacgtgtgcgggggctcccagacacgtgctgggggcaggaatcatagcatttttttgtttgattgttttttgagatggagtctcgctctgtcgcccaggctggagtgcagtggctcaatctcggctcactgcaacctccacctcccgggttcaagcgattctcctgcctcagcctcctgagtagctggaattacaggtgcccgccaccacacccagctaatttttgtatttttttgtcaagacagggattcaccatattggccaggctggtcttgaactcctgacctcaggtgatcctcctgctgcagcctcccaaactgctgggattacaggcgtgagccaccacacccagccaagaatagcattttctttctttctctttttgaggcggagtcttgctctgttgcccaggctggagtgcagtggtgccatctcagtgtaacctccgcctcccggtttcaagcaattcttctgcctcagcctcccgagtagctgggattacaggtgcccgccaccatgcccggctaatttttgtattttcggtggagacagggtttcaccacgttggccaggctggtcttgaactcctgacctcaagtgatccgcccgccttggcctcccaaagtgctgggatgacaggtgtgaaccactgcacccagcccaagaatagcatttttaaaggaaaaaaagcaaggtagaaagatgggtcaaaaccccagcgccccgctgggaggctggtgcccgtgtcgtggcgtgtgtgagatatgtacggaagcgcgaggcggcttccacggctctggctcagggcagcactcacagggcacacggcctcggcggtgtgacgagctgggccgtgggtgcgctgtcctctggggtggggctggccatcctctgttggcgacctagttaacgcccatctccccgcagcctgcctgctccgcttcagcggactctcgctggtctacctgctcttcctgctgctgctgccctggttccccggccccacccgatgcggcctccaaggtaaggccaggggaccctgcccacgctctcagggtgggagggggtgggcattcgtttggggccaaaattcgtacagctttcctcacctttaacagcccggggtggaagatgaggggtcccgaaataaaatttttttttttttttgagacggagtctcgctcagtcgcccaggctggagtgcagtggcgcgatctctgctcactgcaggcttcgcctcccaggttcacgccattctcctgcctcagcctcccgggtagctgggactacaggcgcccgccaccacgcctggcttatttttttttgtatttttagtagagacggggtttcaccgtgatagccaggatggtctcgatctcctgaccttgtgatccgcccgcctcggcctcccaaagtgctgggattacagacgtgagccaccgcgcccggcttttttttttttttttttttttttgagaccgagtctcgctctatctcccaggctggagtgcagtggcacaatcttggctcactgcaacctccgcatcccaggttcaagtaatcctcgcatcccagcctcccaagtagctgcaattacaggtgtgagccaccacgcccagccatcaaagtttcttattttcattgtagaccccaagctaagctcagaatcttttctgatccgtgttgcaggggctgtgaggggcgaggagggtcatgggggtggagtctctgtgtcccttgggaggccacagggagtggatgggccccaactgcccactctctgcaggctccaggcacgtttcctgcctgctgaggctctggcagcctgggagttccagccgcctggaccgccctcccgctgcccgctgtggggttggacctcagttgactttgatccacttgtgcgggggggggggggagctgagaccccccttgggaaccaccttggggtctgagctgggccaggactgtgttgctctcccgtatcctccaaacagagggcggtgaggccacgtgccaagcctgcagcctgggtgacgagggtagcagcaaaccctccatcctgtgacatgtcacctacctgccctgtgggggccatgtccattttgtgcccacgttttaggagagcgcgttttggagcaaacactcagagacctgtccccaaaggccatgggccaaacgtgggtggggccgggccctccgctggtctttgggtttggagggtgaagagccactgaaaggaaggaaggtccccagggagggcaagtgtaggcagcaagagaccttccccagcagagggcagagaggaggccaagcaggaccagggggcgtgactgtggagacaggctcttgggtgccgcccttctgggaggtgctggacgcatcaggctggcagcgtcggggcctgtccatggctacgaggtgtccaccgggctgcgtttttccaggggactctggggaggatctgcttcctcttccagctgctccaggtgcctaccttcctgggcttggggcccctccctccatctccagagccggtggggtggggtcaggatcacaccctgtctctcctgctccctctcccctgcggtaaccctgtggcttcgtcccatctgcctccccggctaatccaggccgacttccctggtttaaggtcagctgttgggcagcccccatttcctctgctgcctggactcgcctctgcatgtgagcttctgcgttcacagattctggggactggggtgcaggcatcattggggtccatcgttctgccagctgcaggtggaaggtcgctctccggcctcgcgacatctggctggaagcatcccagaggctcctcctagctcgtggtgctgtggggtgggcaatggtcttttttatttattttttttgagatggagtctcactctgtcacccaggctggagtgcaatggcacgatctgggctcactgcaacctccgcctcgcgggttcaagcgattctcccgcctcggcctcccgagtagctgggattacaggcgcccaccatcatgcctggctaatttttgtgtttttgtagagacaggggttttaccatgttggccaggctggtcttgaactcctgacctcaggtgatctgcccacctcggccgagactacaggcatgagctaccgtgcttggctttttttttttttttcgagtgggggtcttgcttggttgcccaggctggagagcagtggcatgatcatggctcactgcagcctccacctcctgggctcaagcgatcctcctgccttagcctaccaaagtgctgagattacaggtgtgagtcactgtgcccagcgcaggcactgatcttggatcatgggtagaattcaggggtgcagagaggcattttgggaggggcccagtgcggccgagtgctgggagtcgctggggcccgaggcccaaacccctccaggatgcatggctggggtgggtgggcacccccactcccggtccctatcctgggcctcccctttgctctgtggagccggttctgtctgttcccaggcccctggcgtttcgccgtttgttccgtaaatatttcatgcccagggcgcaattggaaacactttcctttaatcagcagtgggggaaggcaggcgcccagccaggccaggggaggagctggggtgggaagatttggagaggacccgggaggacttccctgcctgagcctcgtcagaggcccttcagagacggagatgctgcccagttttccgggagggagagaggaaagtgtgaggcttgcccgagccgagtgcccggggctttatgatttgtgcagctgctgggcttggcgtggccctggtggaagctctgacgccatctgagccttggtccccttgtaggcgtcagcctgatccttggggggctggaggttgagctcagactgaacagggaggagaggggtaggggctggggctggggcagagggaacagaccctggtgctccaggcagggctgcaggcagagccacagggggtggctcccagagacctgcttgtcatttagggactcagaagccccatcctgccttaggataaaacccacctccaagactgaccctgctgtctggagagagatcaccccccacctcttaccatgccccgtgcagggaggccctgccaccctctccagcttcactggtcccccggctctgccagccttgtgtagtctccatcctctgtctcaaaaggcccctctcgtggccctaccccgcagctcagccctagctgtcgctgggtgggcctcatggctcagcctcaaggcaccctgggtcccttggctggtcccatgcacaccccatggatcaggttccagggggctcccatgcacaccccacggatcagactcagggcaactccacactccccacagaacaatcaggcccagcccttgtccggcaggtgtggggatggtggctatggaccacgcatcaggatgctgccgtggtggggcccctcagcctttgcaggccgtgccggggtccaagggctccggctctgggggaggtccatgctctgtcaaccatccggtctgcaataccctggggcctccccgccccttcctgtttcctcctgagagccctgcaagctggagggggagccccggcccctttttttttttttttttttgagacggagtcttgttctgttgcccaggctggagtgcagtggcgcgatctcaactcactgcaacctccgcctcctgggtttaagtgaaagtgattctcctgcctcagcctcctgagtagctgagattacaggtgcccatcaccacgcctggctaatttttgtattttcagtagaaacagggtttcaccatgttggccaggctggtctcaaactcctgacctgaggtgatccacccacctcggcctcccaaaggtgtgaaccaccacgccaggccccctgcaccttcttctgggtgggcaagagccatgctgagcccctcccctgccatggataggggtggcaagaatagtccattccccatgggctccctccggcaggcagcggatgggttggggcccacacagtggttcaggaaaggctgaagggcggttgccggccagagctgggcgggtccctggcctgagcctcctctcactccctttcccaggatggaaaggccactgtgagctgggtgtgtcctgccaggagggagttggagtcgggggcaggagacccactgggtctcctgggctcctggaagaggcagcagtgggtccctgcggaggtggcctgatccccggctcagcctggttttcccagctttgcatttgggggtgggacctgcagggggagagtgacggggtgggcggggacaggggctgcaggtggaggcacgagaaagccacccgaccccttgaggtcatgctgtttgcgtcggagaagagggccggtgtcagggtgccccctcggcctctgtgtgcacctccccgctccccgccccgtgcaggtcagcagagcctcgatccctctgcacgttccggccccctcccatctccagcagcgtctcttcccggggtgcccctcggactctcagctccctagtctgatccagcccaggcagggagcgggcgtgccacgtggccaggagtggcctccaggcccagctgcggccccttcgaccctgcggagggatcatggcccagctgttctaacatggccagaccaggacactctggccggcccgagaactgaaccgggaaggaggcagggaaaggggagggaggaagacaatggggaagcagtgacatccgagatgtagccagagacggacatcctggactgtcgtgcagggcaaggcgggtgggcgggagccaggtggcctgagagcccctccctgcccaggggtctctggtcaggcagttccttcccgggctgctggatcgtgtgtgcagggaacccgtcagcctggctgcccaagggcccagatgtcctctcagtgcccgggggtccttgacagccccagcaggagccccacgtgcctgtggggcaggccccgcaggtccctctctgtaggactcagaataccttctccaatgccacgtgctctccctgagtgcccagtgccacagagggccccgctggcgaggttacttcaacgtcaggctagagggtgcagcgagcaggactcacagcccaggttcccaggcaggtgtggcaggagcccattccctgggtcggtgttctcatgtcaccccacggtgaccctgctgtacagaggcgggggcgcggggcccctggctggtgccctcctgctgccagacttgtgctctgctgaagaggggctggcgcggcaggtatgagcccggcacggaggtcgtgagcagtgagaagcctggcacctatgggttcggggcagggaggccctggaaggtcctgtcctccgggagccctgcacagcaccccctggtggtggctcctgttcgtgtcggggctgcagcctcccttcctggacggttttccattcctccttcccactctccctgctgctcacccctcccatcctccacaggtcagaggtcatagctgcagggtcagcaggtcagggcctggggcaaccctaggaaggtgtgagtgtgagaagctggtccaaacctgcctcggctgcctggtggtgcggacagggagtcctgggcatccgtgagggctgcttcacggtcaggcttagggatgtgcagggtgacttggacgtgggtcatgagtctttgctccagaaagagggggctgagtgtccaaggccaatcccgagtctgtcacctaacaccatttgtgctcaaaaaactgaacagagtggacacaggccctgagtttgcgccccgaggccgagagagggcagatgtggtggtgacattcaccaccttggacccagacccagatgctacctgtccctgagctccaggaagttgtgagaagggcctgagctgttctgcactttctcgtggccgggcgtggctggtggtgcaggagttgctgccccagggtgagggcccggaagctcctgccagcacgtgccggggtggaaagggaagctgtccacagccctgtcaggactcagaacccggtgggtcaaggactttggtccggacccctgctgaagggtgagctgtccacatgtgcgccgagagcagaggtgaagccagggctcctgagtgcccccagccacagggtgcgcccgcccagcccctgccctgcagccgaaggcctccctgctggggggctgagtccagtggggccacaggcagctgggagcaggacaaggctgccaggcaaccagatggtgctgccgcttcctgccaggtgtgggtgcacagagagagagaggatgccggtctggggcctgacctggtgcacagcaggtgcctgaaatgccagggtggccatggggactgggtaccatgcataggccatgcatcgggatgcaacttctccttgcagcccctcagccccagggaggcagctgcctgccccacttttctccagagccatcatggccctgctcccaccccagccacggctgctcaggggcgctccgcatgctctggtctccatccacctgcagcccccactggggtgaggtggagcttcttgcctctccttgtgtctatttcctctgcttccacaactgaacggtgacaggtatttgctggatgagggagcacaccccaggtggtttcctctgagcctgggaggccttttcctgcctgtgggccccaggcccatcctgctgccacccccaggaggatgcccggctccttgtgacaagagtgaccctcgggaggcgtggggagtggggctggccggcctgcctgatggggtcctgagtccatggcgggtttgcatctcaggcctctgggctctggccgggctgggggctattgtccggctgagcggcctgggctgcggcccctccccgtccccgggaccagcctcacccactcgctctgccgcaggtcacacaggccgcctcctgcgggcattgctgggcctcagcctgctcttcctggtggcccatctcgccctccagatctgcctgcatattgtgccccgcctggaccagctcctgggacccagctgtgagtcgctgagggggcggggtagggatagccatcctgggggtcagggagagggccctgcagtgaccccgagtctcctgggggggttgactcagcctgatttatgtctggcctggatggtccaggtgaaacgctccagggatgaccaggccacggtgctggctgggcagagcctgacctgggttcccccgtctttctctgcaggcagccgctgggagaccctctcgcgacacataggggtcacaaggtaagaccattcctcccacccccaaccagcaagcctcccttggggatttcaggccccaggaagtggggggacccaggagggacagagggggacctggagactcatccacactcccacccacacctggagacccatccacgctcccacccacacctggagacccatccacactctcacccgcacctggagacccatccacactcccacccgcacctggagacccatccacactcccacccgcacctgcagacccatccacactctcacccgcacctggagacccatccacactcccacccgcacctggagacccatccacactcccacccgcacctggagacccatccacactcccacccgcacctggagacccatccacactcacacccacacctgtcctcttggtctgaccgcggctgctccctgctctccgcaggctggacctgaaggacatccccaacgccatccggctggtggcccctgacctgggcatcttggtggtctcctctgtctgcctcggcatctgcgggcgccttgcaaggaacacccggcagagcccacatccacgggagctggtgagggcagctgcgtcacccgtgtgtcagggaggtcattcgagagctgtggtctcagccattttgagggttattttaatctttttaaaacagatgtagacgttttggttgtaagttggtgttaaagagaggaggaagttccaaatcccaccccggggcccagcctgcagttccatccgttcagacctgtttctactcgggctctgcctctagtcagaaacctccacgccccgacatggcatctgtgcccttaggaactcttcacaggggaattatttggggccacgcggtggtggaaacctgcagtgctgggcagtgggtctggctggagagccactgcagaagggctgagaaggggcggccccagcaggccccatgcacttacaggcaaacaggctgtcggcccagagccccagcaggggcctggaccccaggagcgacgggcctgaagcagggcctctgtcctcggagtgggaggcagagtgaactttagctgctacaagacttggaggtccggccccgggaatctctgagctatggccccctcacacggacagggcatgagctggggcctgcgacacccaacgttgactgctcagaccctctcgtccctgcctgggcccacacttgccatccccaggctcagccaggatttatggccacctgggtgtcctggcccacgaactccctgccccgggcacccagcctcctcccacctcaccctcccagtgcccactcgtcagatagctgatgctcgccacgcacatgggcctcaacttctagaggagtcccgagagggaaaggggttccccaagccacacggtaggtcgagtacacctgctcagcctgcagaggcggcctgccctcctgcctgtcctgtcgccaccccatggggcaaggctggtgcccgcatttcagaagtgggaacggggacctggaggtcaagtggcttttccgggcatttgagggggtccagcgctcatgaggactgtgctgctgcctgtcctccaagagacccgcccctccctcgtcagcccctccatgctgatgggggcatggggcatgagcttcctagagtttggctgctgggaaggggctgggtggctggactctggtcatcttcatcttggtgtgatgggagcctgagtgtgcagctgcgccctgggcggccagcgtggacagacttcagagtgagctgggggcaccaggcacctgcaggataccgttccgaaagatctagaagccccatgacccggcctggcagggcccccgggcgaccctcactcccacatatgggcaacacacacacgtgtttgcaggcatgcgacggagtgtgccagccagcccgaggggtgctggccgctagaggagggtgaggggcgtctgcagcatggctgcggcacgtggggcccaagtcagggccgggcctgcccctcggtggcctcacaccccaagtcagggccgggcctgcccctcggtggcctcataccccaagtcagggccgggcctgcccctcggtggcctcacacctgttctctcacagcagctgcctctgttctttccactcccagaaatgctcatttttcacggctctgctcagaagatttcccagggccagggccagggccaggctgtgggtggggtgagcgatggcgccctgcgttctgatccagcctcgcccccagctgctgtgtggtctctgagaggggtgggctcagggcctgggcctctcctgccctgatctccctgttaccctggcctcggagcctcccagcagcccctgcagccctggaggcctgtgaggacaggactggtctggttcatctgtcccgtcaagcccccatcccatttgacagaaggggaataggctccgagaggctgtgacttgcctcggcctgcagagcacggagactgtcagagctggggtggggcctatcgtccagccccacagcctgcggtctcagcccgggcacctggcgcctcagccaccaggagagcccccgagtcacagatggggacactgggccggtggcagccaggccagagccagggcatctgacgacagccgtgttctttccaccacacctggctttccctggtgtttgggaaatggctgtgttctgggaaatctttagtcaggtccagggaaaacaggcccggcaggtctctctccccagccccaggccggcctgtcacttcttctaggcagctggccacctctgtccccccagaggcttggggagggcaggagtaccacccctatcttccaggcagagccacccagaaggctggcaggggtacacaggagaccctggagcctggccatgtccctcaggcccccttggtctctagagaccccccggggtatagacagggccccgctgctccctgggtgcgtggttcggggagatgaggtggtataggacagtctgtggtctgtctgtacctggcaaggtcatcacgtgcctgggcttggcaggacagaccctgggtcttcggccagggtgggagctgctaccaggaaggcctgcaggaactgtgagcttgagtgaggaagtaggaaggtgtcaggcagacctcagggacggctggggcctgtgcccggggaggctgtcctgtggccctcagaggagcagctgtggatgtggccgcctcccacgctcctggctgggcaggtgtgggctggagaggtggcgtcagtgcgatacacctgaccttgcccctgtccgtgaccttggcaggatgatgatgagagggatgtggatgccagcccgacggcagggctgcaggaagcagcaacgctggcccctacacggaggtcacggctggccgctcgtttccgagtcacggcccactggctgctggtggcggctgggcgggtcctggccgtaacactgcttgcactggcaggtacgcaccgaggcagggggcactggcagtcacactgggaggggtcttgggagttccctgatgactgtggagacagcgggacacatggcactggccaggtaccaccctgtgtgcccctgccccgcaggcatcgcccacccctcggccctctccagtgtctacctgctgctcttcctggccctctgcacctggtgggcctgccactttcccatcagcactcggggcttcagcagactctgcgtcgcggtggggtgcttcggcgccggccatctcatctgcctctactgctaccagatgcccttggcacaggctctgctcccgcctgccggcatctgggctaggtaacggcttgccacacagcccctttttcctgccaccctggtcccgcccacctggctcgtctagcccctgtggccccactgcctctggggtggtaggctgtgacgggtcttctctggacagggtgctgggtctcaaggacttcgtgggtcccaccaactgctccagcccccacgcgctggtcctcaacaccggcctggactggcctgtgtatgccagccccggcgtcctcctgctgctgtgctacgccacggcctctctgcgcaagctccgcgcgtaccgcccctccggccaggtgagcacctgccacccatggtgggtgggctgaggccaggccatggggctggtctcaggacctcctgcctctgggtggggtgtggagctggtttgggctcaagacgctggtctctgcagaggaaggaggcggcaaaggggtatgaggctcgggagctggagctagcagagctggaccagtggccccaggaacgggagtctgaccaggtgagcagccaggcaggtggagacgccagcgtggggggcgcccggccagcccgtgcatggctcagcgctgcttgcccacagcacgtggtgcccacagcacccgacaccgaggctgataactgcatcgtgcacgagctgaccggccagagctccgtcctgcggcggcctggtgagtaccgcacactgcaaggtatggctgggtgcggggggcggggcggaggccggtgctgccccctggtggccgcctggcgctctcgcatgctcgcgccgcacctctgcctgccgccccctcgggggcccaggacatccacgggtcggtgtcagtgacccccgagacccccagggcagccgagtggccatgtcactgaccaacccccaagacccccagggcagctgagtggccgcgtcgttgatccccaagaccccatggggggcctccaggtcccccaacccctccccagagaatgtggctatgctgtcttgtgctgttagctctgggagctgctccaggtggcccagtggccccaggaggccgctcgtccagggcaggggctggcctgggaactctgtgttggccacgtcgccttgggagggcctgggggctctttctggctactttctttctttaccctaacccttgattttccattttgcaatgtgtttctgaatgaagcaaatgaagccacggccctggggtgggggtcctgagagtcttcaggtgcgcagagctggaaagggggtcagggccacctttcccaccctttcaaggaaagtgaggcccagagaacggcaggtgctggcagggccatccctgacgctcagggacggtgtcagcccaattgccggagccctcgtgttctgcccatagcccaccgggggcctgtctctcctgctgtgtgcttgcccagggcccagattttagggcatagtcagggtggggaggcctgcagatcaacctgccgaagctgaccgctgtccccacctgcagtgcggcccaagcgggctgagcccagggaggcgtctccgctccacagcctgggccacctcatcatggaccagagctatgtgtgcgcgctcattgccatgatggtaggcggctgtgggggttggggtgggcggccccctctgccgcgcaggtgtggggcatcgcctgggtggggtgcgctgggcagctgtgcagccccctctgccgcgcaggtgtggggcatcgcctgggtggggtgcgctgggcagctgtgcagccccctctgccgcgcaggtgtggggcatcgcctgggtggggtgcgctgggcagctgtgcagccctctctgccgcgcaggtatggagcatcacctaccacagctggctgaccttcgtactgctgctctgggcctgcctcatctggacggtgcgcagccgccaccaactggccatgctgtgctcgccctgcatcctgctgtatgggatgacgctgtgctgcctacgctacgtgtgggccatggacctgcgccctgagctgcccaccaccctgggccccgtcagcctgcgccagctggggctggagcacacccgctacccctgtctggaccttggtgccatggtgagtgtgcaccaccacatccgggggtgcctgggtgcgcagacccatcagggttgtcgtcctgttcaatgtccacttgcccgggggagtggcagcgccaagaaggcagatgtgtctgtctgtccccttctgcccacccagagccagcccagagtagcttctcagtgagcgtttgttgactgaataaacagacaaccttgtgttggcacgggcaccacccctgtgccctgacactgtgtgagcgtgggctctgttggcacgggcaccacccctgtgccccgacactgtgtgtgagcatgggctatgcccattggcacaggcaccacccctgcgcccctgacagtgtgtgtgagcgtgggctctgcccattggcaccatgcacagccctgggtctcagtgacaagctgtgcaggccatgtgttcacagggtgcctgcgtgtccatgtgaaacgggtgccagcatcgtgtctggacacctgtttgcaggccagtgggtctcatcttgtgaaacttgtgagcctgtgtgccaacatatgcacctgtgagcttgtgtgcatatgtgagcacgcatgtgggcaaacatgcactccagcatgtggacatgtgtgcaggtgcgtgcatggatctgtgcccacgtgaactagtgaacccgtgtgtgactctgcgtgtgagcgcaagtgaacccatgcactcatccatggatgtgagagtgtgtgctcgtgtgcctctgagtgggtgtgagcgagagggtgttcggtgcctgtggggaggctgcggtggatgggctggtgccagccgcctgagagctcttgccccctgctataggagggtgctgggtcccccggctgtgggaggggtgctgggccccccggctgactgtgacaccctgcgcttgtcacagttgctctacaccctgaccttctggctcctgctgcgccagtttgtgaaagagaagctgctgaagtgggcagagtctccagctgcgctgacggaggtcaccgtggcagacacaggtgagtggtgggccagaggcgggggttgccctcctgcctgcccgccctgatgccatcgcctgcccctggcttggcccacagagcccacgcggacgcagacgctgttgcagagcctgggggagctggtgaagggcgtgtacgccaagtactggatctatgtgtgtgctggcatgttcatcgtggtcagcttcgccggccgcctcgtggtctacaagattgtctacatgttcctcttcctgctctgcctcaccctcttccaggtggctggggggccgggatgggggctggggcacggaccctccccgcggtcctcaccacccccacctcacccggcaggtctactacagcctgtggcggaagctgctcaaggccttctggtggctcgtggtggcctacaccatgctggtcctcatcgccgtctacaccttccagttccaggacttccctgcctactggcgcaacctcactggcttcaccgacgagcagtgagtccaggctggggcggtggggcaggggcgccgaaaccccgtgcacttccccggggctgcagcggctctgccgggggccgggccggtgctgatgctgcccctccacaggctgggggacctgggcctggagcagttcagcgtgtccgagctcttctccagcatcctggtgcccggcttcttcctcctggcctgcatcctgcagctgcactacttccacaggcccttcatgcagctcaccgacatggagcacgtgtccctgcctggcacgcgcctcccgcgctgggctcacaggtgcggccccgccctccctgtccggccctggagaggtgtagcctcctgggccagggagggagccaggtgggagttggacaggagccacatcttccaccttcagatcccaaggggcatttgctcataccaaggggatggcagtagcgtggaggtcacagggacagtgggcatgagttgcgacacagctgtgcacctgaactggcagctgcagcagaagcggtgccgacagggcttcttccagccccaggaaatgaggggcaggaacccagttgggagatgacattttcggaccctctcccaggcaggatgcagtgagtgggaccccactgctgcgggaggagcagcaggagcatcagcagcagcagcaggaggaggaggaggaggaggaggactccagggacgaggggctgggcgtggccactccccaccaggccacgcaggtgcctgaaggtgggttgggcgggcagagcacagctgccacccagtctgctgtgccatgtcccagctcggggggcgttggcagagtcccctctgggctccagagcctcttcctcacaggggacccgggaatccccgtttgtgccccgcactgaccctcacaccatcacaggggcagccaagtggggcctggtggctgagcggctgctggagctggcagccggcttctcggacgtcctctcacgcgtgcaggtgttcctgcggcggctgctggagcttcacgttttcaagctggtggccctgtacaccgtctgggtggccctgaaggaggtgagtgtggcaggcaactcagcttcccatctggggtggggtcgctctggcctgcccagctggcctccccaagcccagccccacgtgcccactgccctccccaagcccagccccacgtgcccactgccctcaggtgtcggtgatgaacctgctgctggtggtgctgtgggccttcgccctgccctacccacgcttccggcccatggcctcctgcctgtccaccgtgtggacctgcgtcatcatcgtgtgtaagatgctgtaccagctcaaggttgtcaacccccaggagtattccagcaactgcaccgaggtaccggcccccgagggctgggacgggaggaagctccaggcaactctgtattcgcagcccgaccctcctggggcagctgcctcagtgcagtggggccagcaatggagatggaggactctcccctgggggcgccaagggggcttcctggaggcagcatccttcgacctcaactgtggaccaggggcgcactccctgcacacaagggtgtccagtaggggcggagtcccagggtctccggcagtgaggacgggagggccccacccctggacagggagagacagtcaggcatctctgcctgggaccttctcgcacatccctccttctccctggacctctcttcactcccccagcccctgcccgtggtctccctgtttctcaaacacctggtccccttccccgtgaaggtggctccaaggctggcagcccccgtgtccctggctggggagcagtggacctgccccagagctgtggctgtggtgggctccgggcagggccagggggcactgtggcctgggagggggcactgatgcctggcctcttgccagcccttccccaacagcaccaacttgctgcccacggagatcagccagtccctgctgtaccgggggcccgtggaccctgccaactggtttggggtgcggaaagggttccccaacctgggctacatccaggtgagttgaagggctggtgggcggctgggcgggcgagtacccggctgccccctgacccttgccctccgcagaaccacctgcaagtgctgctgctgctggtattcgaggccatcgtgtaccggcgccaggagcactaccgccggcagcaccagctggccccgctgcctgcccaggccgtgtttgccagcggcacccgccagcagctggaccaggatctgctcggctgcctcaagtacttcatcaacttcttcttctacaaattcgggctggaggtgaggcaaggacattgcctccccctggggcagggcttggccttcgggagggagggacggctgcaccgtgcaggcaccgcaagcctggccccacctgggtttgcctgggccacagagggtgggggactcagggccaggcacggcttccctggactcctgtggtgtgtcggtgctgacaacaggcagggggccaagttagatctgctctactgtacagcccacctcctggagcctcagtttcccctgcacgatggcaactgccagccactcctgccctcttgacagcgccgctggccctgtccttgcttgatgcccgcagcctccaggcagggctgctgcaagcctgaggcctgctgggtgggacaagaaagtccctccccccagactcagtgcatccccacaccccgccctctcccctccccagatctgcttcctgatggccgtgaacgtgatcgggcagcgcatgaactttctggtgaccctgcacggttgctggctggtggccatcctcacccgcaggcaccgccaggccattgcccgcctctggcccaactactgcctcttcctggcgctgttcctgctgtaccagtacctgctgtgcctggggatgcccccggccctgtgcattggtgaggggcacgtggcttgggtgggagtgggctttgtggctttgtggatgcccgtgggggtgtttcccgcctgccccagactcctgtccaccctcctagacttagccttggcctcctccagtccctcctctctgctccacatcctacccaggcgccatcacctgcatcctgtctctcgggggcggcctggccccctccaggctctgctgttctcttttccttttttgcccagtattctatcttgaaatatttcaaaccttcaggaaagttgtgagtcacacaaggagcactgcgtcctctccgggccccgtgcgggtcggccgtgatgcctcacacccaagtgctgcctcgagcatgcgtctcctgggtgagggtgtctgagcccacagccccacacccgtggtcccgtctcctggcagtgccatcgtcaaacgtgtcctctgcattcaaacagccccggcctcagcacccttctttgtggccatttggttttcagacgggatctggtctgatgtttgctctagtctcttgtcttgggtctaagccgcccccgcctctcctgtctcttgggaagttccggagggaggccggtagcgttgctgacgccgtgagactggatttgcgtggctgtcctggtgctgcaggtctgctcaaggcacacagcaccctgcggtctgagatggggagtcacatttgtgcacgtggccggctcaggggcgtcccacctgccccacagtggcacccagcctgttggcactggtgggctgtgtggggtcagccttgtggttttacgaaacagactttctctctgctgtctctgtgtgtctgtcagctgggattcccatcaaggacagctgccatttgttactggctgctttccaagaattctgtcatccgcagaccctgggcctcccctctgctgagtgggtcctggcccctccggccacacactgttacatcatctccccgtatttggctgggcatggtggttcacgcctgtgatgccagcactttgggaggctgaggcaggagcatcccttgaggccaggagtttgaaaccactctggtcaacatagcaagaaccctttttttttttttttttttttttgagatggagtcttgctctgtcacccaggctggagtacactggcacaatctcggctcactgcagcctccgcctcccgggttcaagcaattctcctgtctcagcctccctcgtggctaggattacaggcaagcaccaccaggcccggctaatttttgtatttttagtagagacggggtttcaccatcttggccaggctggtcttgaactcctgacctcaggtgatccacccgcctcccaaattacaggcctccctcctgggattacaggcgtgagctgccacgcccggccccgtcttgttttctgctcccaggcgctgctgcctcatcttctgctacccaggcccagccttgtgctcacagccattgctccagggagcccaatcgagttctaggagcgtgaggtttagagcccggggtctgggcgctgggtgtgcctgttgctacagggctgcctcagcctctgggccctccagctcttccttgttgaaacatctgctttcgagcatcaccgaggccagctccccgtctcctgtccacctcttccttgttgaaatacctgctatcaagcgtcacctaggccagctccccttcttctgcctccttccacgcggctgcgccatgcagtcgccatcctgtgagatcagcatgtcctgggttccccaacatcgagggtaactttgtttttgtatcgtgaggttccctctgtggcagatggggctgtgggttcagcatgtcctgggttccccagcatcgagggtcactttgtttttgggtcgcgaggttccctctgtggcagatggggctgtgggttcagcatgtcctgggttccccagcatcgagggtcactttgtttttgtgtcgcgaggttccctctgtggcagatggggctgtgggttcagcatgtcctgggttccccagcatcgagggtcactttgtttttgggtcgcgaggttccctctgtggcagatgggggctgtgggttcagaatgtcctgggttccccagcatcgagggtcactttgtttttgggtcacgaggttccctctgtggcagatggggctgtgggttcagcatgtcctgggttccccagcatcgagggtcactttgtttttgtgtcgcgaggttccctctgtggcagatggggctgtgagatcagcatgtcctgggttccccaacatcgagggtcactttgtttttgggtcgcgaggttccctctgtggcagatggggctgtgggttcagcatgtcctgggttccccagcatcgagggtcactttgtttttgggtcgcgaggttccctctgtggcagatggggctgtgggttcagcatgtcctgggttccccagcatcgagggtcactttgtttttgggtcgcgaggttccctctgtggcagatggggctgtgggttcagaatgtcctgggttccccagcatcgagggtcactttgtttttgggtcgcgaggttccctctgtggcagatggggctgtgggttcagcatgtcctgggttccccagcatcgagggtcactttgtttttgggtcacgaggttccctctgtggcagatggggctgtgggttcagcatgtcctgggttccccaacatcgagggtcactttgtttttgggtcgcgaggttccctctgtggcagatggggctgtgagttcagcatgtcctgggttccccagcatggagggtcactttgtttttgtgtcgcaaggttccctctgtggcagatggggctgtgagttcagcatgtcctgggttccccagcatggagggtcactttgtttttgtgtcgcgaggttccctctgtggcagatggggctgtgagttcagcatgtcctgggttccccagcatggagggtcactttgtttttgtgtcgcgaggttccctctgtggcagatggggctgtgagttcagaatgtcctgggttccccagcatcgagggtcactttgtttttgtgtcgcgaggttccctctgtggcagatggggctgtgagatcagcatgtcctgggttccccaacatcgagggtcactttgtttttgggtcgcgaggttccctctgtggcagatggggctgtgggttcagcatgtcctgggttccccagcatcgagggtcactttgcttttgggtcgcgaggttccctctgtggcagatggggctgtgagttcagcatgtcctgggttccccagcatggagggtcactttgtttttgtgtcgcgaggttccctctgtggcagatggggctgtgggtttcgcagatgcgtggagtcacatccatgccctcagtccttagggaccgaccctccctgcctcacacgcctcccaggaagtgtggccgggggccggcagtgccacggctccctccccagcaggccccggccgctcccatccccagcacgtggtcctatcagaacgccacgtcagcaggactcccagcaggtggcctttaggtctggcttctttcacttggcagagcacactgaggtctgtctaggctgtcgcatggatcccggtcccacgtgctgagcagcgcgttcccagctgtggttgctgcaggttgaacttttcctggctgcaggcgtccgtgcagcttctggccgttgttttcagagctgtcctatcacacgcactgtcctatcatggaatatgacgccgtgtgggccacaactcaggcccagcagcccccacccccgtgctctctggcctcctgctcagttcctttgcccccaggggcttggtgcagagttgaaggaatctgtgtgtgtgaacacacaggacactagagctgtcagttctcgagacaccaggtgtgcgcgaggtgattcccatggaccctgagggctggtgatagactcgggtcaacgggtggggaccgggtgtctcaggccccaggcaggcccggcccttcctgacatgacaccccttcccccagattatccctggcgctggagccgggccgtccccatgaactccgcactcatcaagtggctgtacctgcctgatttcttccgggcccccaactccaccaacctcatcagtgagtgccccccaccacccccgcctctgcagaggaccctcagagtacattcacgcccccaaatctgctcacaagtgtgcacacaggcgtgcacgggcggaggtgtggtcaggcacatggcggcctgcaggccctgacctcgcacgcacgcacgcagacctcagcctgtgtgcacggcagcccttgtgcagatgccctcacaccggggctcccccagggacacccggccactcacccaggcagacgtgtgtccgctcccagcggctgcacgccgacaggcctggggtgggaggtgggatttatgcgccgtgcccacctcgtgtgggtccccgtgtggcacagcggcggctcctgtgtcctgcaggcgactttctcctgctgctgtgcgcctcccagcagtggcaggtgttctcagctgagcgcacagaggagtggcagcgcatggctggcgtcaacaccgaccgcctggagccgctgcggggggagcccaaccccgtgcccaactttatccactgcaggtgggttccacgtcaccctccacggggaaccttctgggaggggtggccggggcgcccgccctgacgctccggcctggcaggtcctaccttgacatgctgaaggtggccgtcttccgatacctgttctggctggtgctggtggtggtgtttgtcacgggggccacccgcatcagcatcttcgggctgggctacctgctggcctgcttctacctgctgctcttcggcacggccctgctgcagagggacacacgggcccgcctcgtgctgtgggactgcctcattctgtacaacgtcaccgtcatcatctccaagaacatgctgtcggtgagcctccggcccccccgcacccaccgccctggggccccgctggccccgctgaccctgctctcccccagctcctggcctgcgtcttcgtggagcagatgcagaccggcttctgctgggtcatccagctcttcagccttgtatgcaccgtcaagggctactatgaccgtgagtggccaggacggtggcgggggagggcgtggggaagccccctgctcctgggccctgggcctgacccttgccggtgcctgccttgcagccaaggagatgatggacagagaccaggactgcctgctgcctgtggaggaggctggcatcatctgggacagcgtctgcttcttcttcctgctgctgcagcgccgcgtcttccttagccattactacctgcacgtcagggccgacctccaggccaccgccctgctagcctccaggcaagcttgggcccagacacagcccagagctcccgtcttggggctgggagggggcaatgggaggttcctcactgtctcaggccccggcccgtggagggcaggctctgccactctgtgacatgggcgtgtcatctagagggagaatgaaggccggcagatccccggcaccatcacactctgccccagtgctgggtctgtcagagaccacaggctgcagtgctgacggtggctggtgtctcacccccagccaactttcccactaagggctaagtttctccaccagcgggagggccactgtgtggtgtcacgactgccccagggaggggttctggcttggggccagctttgccttcttccctgcagctgtggtggggtgggtgccaccagacgcccctgcatctgtacggcagaagggcctgtcctcgccgcagacagcacggagggtgggggcagcagatgcctcccccgtgggtgcctcttgtccagcgtgggcagagaggagcaggctgagctgtcccgggctgagcggggagcggcggctgcccatgttgctggggtcgagtgcctggtgctcacaccccatccccgcctccctacaggggcttcgccctctacaacgctgccaacctcaagagcattgactttcaccgcaggatagaggagaagtccctggcccagctgaaaagacagtaggtgcctctggggcggggactccccggctcctccccccaatgctcagcataccccacctttccccaccacaggatggagcgtatccgtgccaagcaggagaagcacaggcagggccgggtggaccgcagtcgcccccaggacaccctgggccccaaggaccccggcctggagccaggtgagtgcagctggagtcgggcacccagggccccgtgtccagcatgtctgtgcctgctggcgtgtgctgcgtctgtgcccatgtgacgtcccacagggctcccagcccgcctgtcctgtccgcatgatcaccctctgtctggcaggccccatggccgccctgtgactgtccgtccacgcacatgggctctgagccccatggccccacacggcccccgtcactgtgggtgtccgtgtctgtctccacctatcctgtctccaagacgggagcactcacagccccgacccctcctggtggcttgactgctgcctcatgctcaccctgcccctccacagggcccgacagtccagggggctcctccccgccacggaggcagtggtggcggccctggctggaccacgccacaggtacccccaattaggccgcctgtggccaccctctcaggccctctgtgcccccatctgtcctctgcctggcctgctatcttcccctcccttcccccgactcccaggccctgagcgtcaggacgtgctcaggcctcctgggtcggggggtgcctcactggctgcagacccctgggctgactatgtcctctcctggctatgccccagcccttccaacagtgggagtctcggagcttgccccgatgacacatggtggtcgagcagcgatctcacctgggacccagcagcactgcgttattctgtttttgtttctttttgagatggagtctcgctctgtcactgcaggctggagtgcagtggcatgatctcagctcactgcaatctctacctcccgggttcaagtgatcctcctgcctcagcctcccaagtaactgagactacaagcatgtgccccactccaggccttttttttttttttttggagacggtgtcttgccctgtcgcccaggctacagtgcaatggcgtgattgcggctcactacaacccccacctcccaggttcaaaggattctcctgcctcagcctcccaagtagctgggattacaggtgcccgccaccacgcccagctaattttcgtatttttagtagagatggggtttcaccatattggccaggctggtctcgaacctctgacttcaggtgatccgcccgcctcagcctcccacagtgctgggattacaggcgtcagccaccgtgcccggcctgttctgtttttctaactctcacacagcctcctgggttttccccggtcctctgcagtcggcccactctgcaccccagcccgcgctggctctgctcctcagctgccctgcccacctctgtcttgtcccaccgcgctggcctgtgtcttgtgcctgcactgctcccggctactccgcatgggaagggtggctctcgggccttggcccatgcaggcggagggggtctggctgggagtctccctgcatggaaggctggctctcagtgctgcctgcccacagtcatccactccggggactacttcctgtttgagtccgacagtgaggaagaggaggaggctgttcctgaagacccgaggccgtcggcacagagtgccttccaggtgaggtgggagagccccgtcggccccactccaaccacagagcttgtggtcctggaccagggcagcatagagggtgtcagatgcccccagggcctgggagccgagctcctccacctccagttagcccaccccgccccatccaggcctcccaagtcccatgggaaaccaggctacagggacatgggtcatgtgtagcctgctgccccacggtcttggctctgaccacccaggttctggtggctgcccgtggcctgacctgtgagaccggcccaacacctttgtgctggccgcctggctgtcctgggtccatctttgggcccctggctcttggtgttagaccagcccacccaactcctgaatgggtgggagtcttcccccacagcccctcagggtccccatccgggaggggctcagggacacggaggtccctgggagacacagagcagggatctggatctggcgcccggcttgcccaaccccagcttcccgcctgggtctgatggctcgggaggccgggtcctaacccgggggctggccgacagctggcgtaccaggcatgggtgaccaacgcccaggcggtgctgaggcggcggcagcaggagcaggagcaggcaaggcaggaacaggcaggacagctacccacaggtgagctggggggcgtggggactctgaggggaagccgcgggactgccagtcactcaccagcatcctgtgcccaggaggtggtcccagccaggaggtggagccagcagagggccccgaggaggcagcggcaggtacgtgggcccggggctggggagtgggaggtctctcttggccccacaggctgcccctccagcgccccctcccgccctcccgcaggccggagccatgtggtgcagagggtgctgagcacggcgcagttcctgtggatgctggggcaggcgctagtggatgagctgacacgctggctgcaggagttcacccggcaccacggcaccatgagcgacgtgctgcgggcagagcgctacctcctcacacaggagctcctgcaggtgagcctgcccgtgcaccacgctcgtccctgctctgcctgactacgcccctgcctgcttaacagcctagtcccgcgcccactgcacgaaaccccgtgtggggacaagagctggacgcagccctgagccccctgctgtgccctgcagggcggcgaagtgcacaggggcgtgctggatcagctgtacacaagccaggccgaggccacgctgccaggccccaccgaggcccccaatgccccaagcaccgtgtccaggtaggtgcgggggtgacccgagccccagctgctgcccctggtgtgtgggcatcgcctagccatccccgaccctcgccattcccttgtaccccaaaggaccgtgggcactttccaccctgaccctccctgtagcctggggtcaggccatagagcaggattctctgtgactcggcttccctccccagtgggctgggcgcggaggagccactcagcagcatgacagacgacatgggcagccccctgagcaccggctaccacacgcgcagtggcagtgaggaggcagtcaccgaccccggggagcgtgaggctggtgcctctctgtaccagggactgatgcggacggccagcgagctgctcctggacaggtgggggcgggacgcgcacaacaccagcctcaccatggccctcggggagcagccgaacaggggcaggagactgactgtgaccggcaacagatcgggccgtcatgccttcgggcagtcccagactcccccaaacacgcgggtctccctgtaggcgcctgcgcatcccagagctggaggaggcagagctgtttgcggaggggcagggccgggcgctgcggctgctgcgggccgtgtaccagtgtgtggccgcccactcggagctgctctgctacttcatcatcatcctcaaccacatggtcacggcctccgccggctcgctggtgctgcccgtgctcgtcttcctgtgggccatgctgtcgatcccgaggcccagcaagcgcttctggatgacggccatcgtcttcaccgaggtgggccgaggccgcgggggagggggcgcccggcccaccgcgccgtgaccctccccgcgtgctgagccccctcccccacagatcgcggtggtcgtcaagtacctgttccagtttgggttcttcccctggaacagccacgtggtgctgcggcgctacgagaacaagccctacttcccgccccgcatcctgggcctggagaagactgacggctacatcaagtacgacctggtgcagctcatggcccttttcttccaccgctcccagctgctggtgagtgtgagccttggctggcaatgcggggctgggcaggccctctgggcacctgtgctctccaccagggaggcaaggccccctcaccacaccctcccgcccctcagtgctatggcctctgggaccatgaggaggactcaccatccaaggagcatgacaagagcggcgaggaggagcagggagccgaggaggggccaggggtgcctgcggccaccaccgaagaccacattcaggtggaagccagggtcggacccacggacgggaccccagaaccccaagtggagctcaggccccgtgatacgaggcgcatcagtctacgttttagaagaaggaagaaggagggcccagcacggaaaggagcggcagccatcggtataagcgccctgcctcacaacctcctgcctacccagttttctgagtggggctactgcagggagggtctttctcagatgagacggccaagcccagtgcgaggcccacctggatcccaggaaggtgccacttctgagccacagctcccggctctgcctacagagccgtccctgactgctgcccccggggatgctccccacgtgtagggtgactgttggcctgggctggcccctcacagttgccccagacagaggacacagccccagctgtctccttgccagtgacactgggagctttcctgtgctccgtctgcttgtctgtcaaacagggagaatgccagcctcttagggtggtcaggagccatgagccaggcccagtccccagggggcccaggcagaagtcagcttttccctacagaagctgaggacagggaggaagaagagggggaggaagagaaagaggcccccacggggagagagaagaggccaagccgctctggaggaagagtaagggcggccgggcggcggctgcagggcttctgcctgtccctgtgagtgatggcggccgggggcagctggggagtgggggtggggaggcgggtactgggcccaggctgagcgcccccttccgcagggcccagggcacatatcggccgctacggcgcttcttccacgacatcctgcacaccaagtaccgcgcagccaccgacgtctatgccctcatgttcctggctgatgttgtcgacttcatcatcatcatttttggcttctgggcctttggggtgagccaggcccgggacccaaacccagtgtacgcagagctcagcagccacccacatcccctgggcttggctccccctgacctgtgctctcctggccacagaagcactcggcggccacagacatcacgtcctccctatcagacgaccaggtacccgaggctttcctggtcatgctgctgatccagttcagtaccatggtggttgaccgcgccctctacctgcgcaagaccgtgctgggcaagctggccttccaggtggcgctggtgctggccatccacctatggatgttcttcatcctgcccgccgtcactgagaggtgggcccacgcgtgggggcgctcggtctccaggggcggggcagtgcaggctgggggccctgcggggctgtttctgatggggtccttgacctggccatcccgccccaggatgttcaaccagaatgtggtggcccagctctggtacttcgtgaagtgcatctacttcgccctgtccgcctaccagatccgctgcggctaccccacccgcatcctcggcaacttcctcaccaagaagtacaatcatctcaacctcttcctcttccaggggtgagtgcaggtccgccggggtgggggtcacggcccgggcatgagggagcccacctgacgggaaccctggctgtgggcaggttccggctggtgccgttcctggtggagctgcgggcagtgatggactgggtgtggacggacaccacgctgtccctgtccagctggatgtgtgtggaggacatctatgccaacatcttcatcatcaaatgcagccgagagacagagaaggtgcctgggcccagggcgggggccgggacaagggccagggatatgccctctccctaagacagaggcactgctgccacgagaacccgtggtgctggaggccctcccagggctcggagcccatggggacatgaggcgagcccacccactagctgatcacgaggccagtgatcttggcagctgcgagtgagtgctgggcgcagaagtgggcagcggagttggtcctgttccaggcaggctggcagcagagcagggcctggtgcagggaggaccggacagccactgtttgctgcattcttgtttaatggcctttctcagagagaattcgtgcgtcagaccactcccccacgtaaaaagtacaactcaggggtttctagtggattcacagttgagcatctgccttctcaccacttcaaaaagaaaccccgggccgggcacagcggctcacccctatcatcccagcactgtaagagacccaggagggaggtactgctcaaggccaggagttcaagatctgcacggccacaagcgagaccctgcctcagcaaatgtaaaaataaaacaattagctggcaatggcagctcatgcctatggtcccagcactttgggaggccaaaggaggaggatcagttgaggccaggagttttaagaccagcctgggcaacatagtgagtgagactctctctacaaaaaaataaacgttagctgggtgtgatggtgcacacttgtgctcccagctactctggaggctgaggtgggaggatggcttgaggccaggagtacagggctgcattaagcctgatcacaccactgcactccagcttgggcaacagagtgagaccctgtctctaaaaaagtaaaaagaagaaacccagtgcccattggctgtcactcggtttcccctcccctggcccctagtaaccccttgtctaggtcctggttctatgagatttgcctacagtggatatttcatgaaaacaggctcagacagcgtttgtccttttgtaatcagctttccttgctcagcatggtgtctctgaggtccacccacgtggcagtatggccttcctgtttatgggcaaatgatattctgtggcatggatggaccacaacatgctcatctgttgatgggctgttgcccgtgatgctgccaggcacgccggtgtacacgtctgtgtgcccgtgcccctggtcctgtggctgcacgccagggccggaagtgctggtggtggtttccatcatgaggagctgctggttttccatagcagctccaccatctaaggttcccaccaccaacacgaggttgcggtttctccacatcctcaacaacctgttactatgtcttttttgttctggccatgctgctgaacgggtggcttgctgtgggctcttctcagttccctgttgaccgacgctgagcgtcttttcatgtgcttggccatttgtgtatcttctctggggaaatgtctattcaaatcctttctccatagtttagttgggcttttgagataggatctcaggctgaagtgcagtggcatgaccttcactcactgtagcctctgcctcccaggttcaagcgattctcccacctcagcctcccgagtagctgggactacaggtgtgcaccaccaggcctggctagtcttttgtatttttggccaggttcgtctcaaactcctgacctcaaagtgctgggatgacaagtgtgagccgccacacccagcagttgggttgttttttattagagttttttctgtttttctgcagatacattggctagaaatgactgaattggaagaattctctgtattctctggttgctagaaccttatcaattaaaatttgcagaaaatttctccaattctatggactgtctcttaaattttcttggtgtctttggaagcacaaagtatttattttggtaatatctggtttactttgtttccttcgccaaatccaggttcatgaagatttgcccgttttcttctaaaagttctatagttttagctctgaagtttcgctctttgatccactttgaggtaaattttggcacatggtatgaggcaggagttgcgtttcattctcctgcctggggcggtgcctgcaccgtgttgaaaaaggttgtccgttcccactgaacggtcacagctcccttgtctaagatcaacgacccctgaacatgagggttccaactggactcttagttctactccactggcctgtgtctgcccaccattactaccgctgtgccatactgaggtcaggctggggcttttctgggctgctgggtgagctggagaatgcggttgtgtgacccgcaggaagggcagagctgagcgtatgacctgtgtcgttcccctccagaaatacccgcagcccaaagggcagaagaagaagaagatcgtcaagtacggcatgggtggcctcatcatcctcttcctcatcgccatcatctggttcccactgctcttcatgtcgctggtgcgctccgtggttggggttgtcaaccagcccatcgatgtcaccgtcaccctgaagctgggcggctatgaggtgagcatgtgtgggtccgcctgtccattcccatcccctgggggttctggccaaggtggtgcaccacccccagccgctcctccacgctcatcttcgtggccccgtgtccccgtgcctgccccagccgctgttcaccatgagcgcccagcagccgtccatcatccccttcacggcccaggcctatgaggagctgtcccggcagtttgacccccagccggtaagtggcctctgccctgtgaaagctggtgtggggaggcggctgcagtcactgagggtgtcacttgtacccagctggccatgcagttcatcagccagtacagccctgaggacatcgtcacggcgcagattgagggcagctccggggcgctgtggcgcatcagtccccccagccgtgcccagatgaagcgggagctctacaacggcacggccgacatcaccctgcgcttcacctggaacttccagaggttcgtcctggacttggggcagtgcctgggtgggtggacccactacagtgggtcacgctgtgttcccacccccagggacctggcgaagggaggcactgtggagtatgccaacgagaagcacatgctggccctggcccccaacagcactgcacggcggcagctggccagcctgctcgagggcacctcggaccagtctgtgtgagtgaagggcccgggtggtgggcaggagggctgtgccaggttggctgggccaggcctgacctgccagcacctccctgcagggtcatccctaatctcttccccaagtacatccgtgcccccaacgggcccgaagccaaccctgtgaagcagctgcagcccagtgagtatgggcgtgggggttgggggaggctagagaggggtgacctgcggcctcaacgatcttctccctccatcccagatgaggaggccgactacctcggcgtgcgtatccagctgcggagggagcagggtgcgggggccaccggcttcctcgaatggtgggtcatcgagctgcaggagtgccggaccgactgcaacctgctgcccatggtcattttcagtgacaaggtcagcccaccgagcctcggcttcctggctggctacgggtgagtgagtggctgggggggcaccccgcagctcggggggctccgggcggccccaggactcaccagcttcccccgcagcatcatggggctgtacgtgtccatcgtgctggtcatcggcaagttcgtgcgcggattcttcagcgagatctcgcactccattatgttcgaggagctgccgtgcgtggaccgcatcctcaagctctgccaggacatcttcctggtgcgggagactcgggagctggagctggaggaggagttgtacgccaagctcatcttcctctaccgctcaccggagaccatgatcaagtggactcgtgagaaggagtaggagctgctgctggcgcccgagagggaaggagccggcctgctgggcagcgtggccacaaggggcggcactcctcaggccgggggagccactgccccgtccaaggccgccagctgtgatgcatcctcccggcctgcctgagccctgatgctgctgtcagagaaggacactgcgtccccacggcctgcgtggcgctgccgtcccccacgtgtactgtagagttttttttttaattaaaaaatgttttatttatacaaatggacaatcaga

SEQ ID NO: 2 - DNA, 8089 bp, Homo sapiens
  source 1..8089: mol_type = other DNA
gggagccgccgtccggcccagctcggccccagtgagccgagcgctgcgctccgccgaggggcagggcggtcgcctgagcgagcgcgggcccgggacgtcggcaccggcggggcggccgaaggagaaggaggaagaggagaaggcggcgcgcgggtccccgcgggtcagccatggcgcgccggccccggggcccccgcaccgccccatagcgccgcggcgtccgctcggtctgggccgggccctgggccctccagccatggagccgcacgtgctcggcgcggtcctgtactggctgctgctgccctgcgcgctgctggctgcctgcctgctccgcttcagcggactctcgctggtctacctgctcttcctgctgctgctgccctggttccccggccccacccgatgcggcctccaaggtcacacaggccgcctcctgcgggcattgctgggcctcagcctgctcttcctggtggcccatctcgccctccagatctgcctgcatattgtgccccgcctggaccagctcctgggacccagctgcagccgctgggagaccctctcgcgacacataggggtcacaaggctggacctgaaggacatccccaacgccatccggctggtggcccctgacctgggcatcttggtggtctcctctgtctgcctcggcatctgcgggcgccttgcaaggaacacccggcagagcccacatccacgggagctggatgatgatgagagggatgtggatgccagcccgacggcagggctgcaggaagcagcaacgctggcccctacacggaggtcacggctggccgctcgtttccgagtcacggcccactggctgctggtggcggctgggcgggtcctggccgtaacactgcttgcactggcaggcatcgcccacccctcggccctctccagtgtctacctgctgctcttcctggccctctgcacctggtgggcctgccactttcccatcagcactcggggcttcagcagactctgcgtcgcggtggggtgcttcggcgccggccatctcatctgcctctactgctaccagatgcccttggcacaggctctgctcccgcctgccggcatctgggctagggtgctgggtctcaaggacttcgtgggtcccaccaactgctccagcccccacgcgctggtcctcaacaccggcctggactggcctgtgtatgccagccccggcgtcctcctgctgctgtgctacgccacggcctctctgcgcaagctccgcgcgtaccgcccctccggccagaggaaggaggcggcaaaggggtatgaggctcgggagctggagctagcagagctggaccagtggccccaggaacgggagtctgaccagcacgtggtgcccacagcacccgacaccgaggctgataactgcatcgtgcacgagctgaccggccagagctccgtcctgcggcggcctgtgcggcccaagcgggctgagcccagggaggcgtctccgctccacagcctgggccacctcatcatggaccagagctatgtgtgcgcgctcattgccatgatggtatggagcatcacctaccacagctggctgaccttcgtactgctgctctgggcctgcctcatctggacggtgcgcagccgccaccaactggccatgctgtgctcgccctgcatcctgctgtatgggatgacgctgtgctgcctacgctacgtgtgggccatggacctgcgccctgagctgcccaccaccctgggccccgtcagcctgcgccagctggggctggagcacacccgctacccctgtctggaccttggtgccatgttgctctacaccctgaccttctggctcctgctgcgccagtttgtgaaagagaagctgctgaagtgggcagagtctccagctgcgctgacggaggtcaccgtggcagacacagagcccacgcggacgcagacgctgttgcagagcctgggggagctggtgaagggcgtgtacgccaagtactggatctatgtgtgtgctggcatgttcatcgtggtcagcttcgccggccgcctcgtggtctacaagattgtctacatgttcctcttcctgctctgcctcaccctcttccaggtctactacagcctgtggcggaagctgctcaaggccttctggtggctcgtggtggcctacaccatgctggtcctcatcgccgtctacaccttccagttccaggacttccctgcctactggcgcaacctcactggcttcaccgacgagcagctgggggacctgggcctggagcagttcagcgtgtccgagctcttctccagcatcctggtgcccggcttcttcctcctggcctgcatcctgcagctgcactacttccacaggcccttcatgcagctcaccgacatggagcacgtgtccctgcctggcacgcgcctcccgcgctgggctcacaggcaggatgcagtgagtgggaccccactgctgcgggaggagcagcaggagcatcagcagcagcagcaggaggaggaggaggaggaggaggactccagggacgaggggctgggcgtggccactccccaccaggccacgcaggtgcctgaaggggcagccaagtggggcctggtggctgagcggctgctggagctggcagccggcttctcggacgtcctctcacgcgtgcaggtgttcctgcggcggctgctggagcttcacgttttcaagctggtggccctgtacaccgtctgggtggccctgaaggaggtgtcggtgatgaacctgctgctggtggtgctgtgggccttcgccctgccctacccacgcttccggcccatggcctcctgcctgtccaccgtgtggacctgcgtcatcatcgtgtgtaagatgctgtaccagctcaaggttgtcaacccccaggagtattccagcaactgcaccgagcccttccccaacagcaccaacttgctgcccacggagatcagccagtccctgctgtaccgggggcccgtggaccctgccaactggtttggggtgcggaaagggttccccaacctgggctacatccagaaccacctgcaagtgctgctgctgctggtattcgaggccatcgtgtaccggcgccaggagcactaccgccggcagcaccagctggccccgctgcctgcccaggccgtgtttgccagcggcacccgccagcagctggaccaggatctgctcggctgcctcaagtacttcatcaacttcttcttctacaaattcgggctggagatctgcttcctgatggccgtgaacgtgatcgggcagcgcatgaactttctggtgaccctgcacggttgctggctggtggccatcctcacccgcaggcaccgccaggccattgcccgcctctggcccaactactgcctcttcctggcgctgttcctgctgtaccagtacctgctgtgcctggggatgcccccggccctgtgcattgattatccctggcgctggagccgggccgtccccatgaactccgcactcatcaagtggctgtacctgcctgatttcttccgggcccccaactccaccaacctcatcagcgactttctcctgctgctgtgcgcctcccagcagtggcaggtgttctcagctgagcgcacagaggagtggcagcgcatggctggcgtcaacaccgaccgcctggagccgctgcggggggagcccaaccccgtgcccaactttatccactgcaggtcctaccttgacatgctgaaggtggccgtcttccgatacctgttctggctggtgctggtggtggtgtttgtcacgggggccacccgcatcagcatcttcgggctgggctacctgctggcctgcttctacctgctgctcttcggcacggccctgctgcagagggacacacgggcccgcctcgtgctgtgggactgcctcattctgtacaacgtcaccgtcatcatctccaagaacatgctgtcgctcctggcctgcgtcttcgtggagcagatgcagaccggcttctgctgggtcatccagctcttcagccttgtatgcaccgtcaagggctactatgaccccaaggagatgatggacagagaccaggactgcctgctgcctgtggaggaggctggcatcatctgggacagcgtctgcttcttcttcctgctgctgcagcgccgcgtcttccttagccattactacctgcacgtcagggccgacctccaggccaccgccctgctagcctccaggggcttcgccctctacaacgctgccaacctcaagagcattgactttcaccgcaggatagaggagaagtccctggcccagctgaaaagacagatggagcgtatccgtgccaagcaggagaagcacaggcagggccgggtggaccgcagtcgcccccaggacaccctgggccccaaggaccccggcctggagccagggcccgacagtccagggggctcctccccgccacggaggcagtggtggcggccctggctggaccacgccacagtcatccactccggggactacttcctgtttgagtccgacagtgaggaagaggaggaggctgttcctgaagacccgaggccgtcggcacagagtgccttccagctggcgtaccaggcatgggtgaccaacgcccaggcggtgctgaggcggcggcagcaggagcaggagcaggcaaggcaggaacaggcaggacagctacccacaggaggtggtcccagccaggaggtggagccagcagagggccccgaggaggcagcggcaggccggagccatgtggtgcagagggtgctgagcacggcgcagttcctgtggatgctggggcaggcgctagtggatgagctgacacgctggctgcaggagttcacccggcaccacggcaccatgagcgacgtgctgcgggcagagcgctacctcctcacacaggagctcctgcagggcggcgaagtgcacaggggcgtgctggatcagctgtacacaagccaggccgaggccacgctgccaggccccaccgaggcccccaatgccccaagcaccgtgtccagtgggctgggcgcggaggagccactcagcagcatgacagacgacatgggcagccccctgagcaccggctaccacacgcgcagtggcagtgaggaggcagtcaccgaccccggggagcgtgaggctggtgcctctctgtaccagggactgatgcggacggccagcgagctgctcctggacaggcgcctgcgcatcccagagctggaggaggcagagctgtttgcggaggggcagggccgggcgctgcggctgctgcgggccgtgtaccagtgtgtggccgcccactcggagctgctctgctacttcatcatcatcctcaaccacatggtcacggcctccgccggctcgctggtgctgcccgtgctcgtcttcctgtgggccatgctgtcgatcccgaggcccagcaagcgcttctggatgacggccatcgtcttcaccgagatcgcggtggtcgtcaagtacctgttccagtttgggttcttcccctggaacagccacgtggtgctgcggcgctacgagaacaagccctacttcccgccccgcatcctgggcctggagaagactgacggctacatcaagtacgacctggtgcagctcatggcccttttcttccaccgctcccagctgctgtgctatggcctctgggaccatgaggaggactcaccatccaaggagcatgacaagagcggcgaggaggagcagggagccgaggaggggccaggggtgcctgcggccaccaccgaagaccacattcaggtggaagccagggtcggacccacggacgggaccccagaaccccaagtggagctcaggccccgtgatacgaggcgcatcagtctacgttttagaagaaggaagaaggagggcccagcacggaaaggagcggcagccatcgaagctgaggacagggaggaagaagagggggaggaagagaaagaggcccccacggggagagagaagaggccaagccgctctggaggaagagtaagggcggccgggcggcggctgcagggcttctgcctgtccctggcccagggcacatatcggccgctacggcgcttcttccacgacatcctgcacaccaagtaccgcgcagccaccgacgtctatgccctcatgttcctggctgatgttgtcgacttcatcatcatcatttttggcttctgggcctttgggaagcactcggcggccacagacatcacgtcctccctatcagacgaccaggtacccgaggctttcctggtcatgctgctgatccagttcagtaccatggtggttgaccgcgccctctacctgcgcaagaccgtgctgggcaagctggccttccaggtggcgctggtgctggccatccacctatggatgttcttcatcctgcccgccgtcactgagaggatgttcaaccagaatgtggtggcccagctctggtacttcgtgaagtgcatctacttcgccctgtccgcctaccagatccgctgcggctaccccacccgcatcctcggcaacttcctcaccaagaagtacaatcatctcaacctcttcctcttccaggggttccggctggtgccgttcctggtggagctgcgggcagtgatggactgggtgtggacggacaccacgctgtccctgtccagctggatgtgtgtggaggacatctatgccaacatcttcatcatcaaatgcagccgagagacagagaagaaatacccgcagcccaaagggcagaagaagaagaagatcgtcaagtacggcatgggtggcctcatcatcctcttcctcatcgccatcatctggttcccactgctcttcatgtcgctggtgcgctccgtggttggggttgtcaaccagcccatcgatgtcaccgtcaccctgaagctgggcggctatgagccgctgttcaccatgagcgcccagcagccgtccatcatccccttcacggcccaggcctatgaggagctgtcccggcagtttgacccccagccgctggccatgcagttcatcagccagtacagccctgaggacatcgtcacggcgcagattgagggcagctccggggcgctgtggcgcatcagtccccccagccgtgcccagatgaagcgggagctctacaacggcacggccgacatcaccctgcgcttcacctggaacttccagagggacctggcgaagggaggcactgtggagtatgccaacgagaagcacatgctggccctggcccccaacagcactgcacggcggcagctggccagcctgctcgagggcacctcggaccagtctgtggtcatccctaatctcttccccaagtacatccgtgcccccaacgggcccgaagccaaccctgtgaagcagctgcagcccaatgaggaggccgactacctcggcgtgcgtatccagctgcggagggagcagggtgcgggggccaccggcttcctcgaatggtgggtcatcgagctgcaggagtgccggaccgactgcaacctgctgcccatggtcattttcagtgacaaggtcagcccaccgagcctcggcttcctggctggctacggcatcatggggctgtacgtgtccatcgtgctggtcatcggcaagttcgtgcgcggattcttcagcgagatctcgcactccattatgttcgaggagctgccgtgcgtggaccgcatcctcaagctctgccaggacatcttcctggtgcgggagactcgggagctggagctggaggaggagttgtacgccaagctcatcttcctctaccgctcaccggagaccatgatcaagtggactcgtgagaaggagtaggagctgctgctggcgcccgagagggaaggagccggcctgctgggcagcgtggccacaaggggcggcactcctcaggccgggggagccactgccccgtccaaggccgccagctgtgatgcatcctcccggcctgcctgagccctgatgctgctgtcagagaaggacactgcgtccccacggcctgcgtggcgctgccgtcccccacgtgtactgtagagttttttttttaattaaaaaatgttttatttatacaaatggacaatcaga

SEQ ID NO: 3 - DNA, 8089 bp, Homo sapiens; identical to SEQ ID NO: 2
  source 1..8089: mol_type = other DNA

SEQ ID NO: 4 - protein, 2521 aa, Homo sapiens
MEPHVLGAVLYWLLLPCALLAACLLRFSGLSLVYLLFLLLLPWFPGPTRCGLQGHTGRLLRALLGLSLLFLVAHLALQICLHIVPRLDQLLGPSCSRWETLSRHIGVTRLDLKDIPNAIRLVAPDLGILVVSSVCLGICGRLARNTRQSPHPRELDDDERDVDASPTAGLQEAATLAPTRRSRLAARFRVTAHWLLVAAGRVLAVTLLALAGIAHPSALSSVYLLLFLALCTWWACHFPISTRGFSRLCVAVGCFGAGHLICLYCYQMPLAQALLPPAGIWARVLGLKDFVGPTNCSSPHALVLNTGLDWPVYASPGVLLLLCYATASLRKLRAYRPSGQRKEAAKGYEARELELAELDQWPQERESDQHVVPTAPDTEADNCIVHELTGQSSVLRRPVRPKRAEPREASPLHSLGHLIMDQSYVCALIAMMVWSITYHSWLTFVLLLWACLIWTVRSRHQLAMLCSPCILLYGMTLCCLRYVWAMDLRPELPTTLGPVSLRQLGLEHTRYPCLDLGAMLLYTLTFWLLLRQFVKEKLLKWAESPAALTEVTVADTEPTRTQTLLQSLGELVKGVYAKYWIYVCAGMFIVVSFAGRLVVYKIVYMFLFLLCLTLFQVYYSLWRKLLKAFWWLVVAYTMLVLIAVYTFQFQDFPAYWRNLTGFTDEQLGDLGLEQFSVSELFSSILVPGFFLLACILQLHYFHRPFMQLTDMEHVSLPGTRLPRWAHRQDAVSGTPLLREEQQEHQQQQQEEEEEEEDSRDEGLGVATPHQATQVPEGAAKWGLVAERLLELAAGFSDVLSRVQVFLRRLLELHVFKLVALYTVWVALKEVSVMNLLLVVLWAFALPYPRFRPMASCLSTVWTCVIIVCKMLYQLKVVNPQEYSSNCTEPFPNSTNLLPTEISQSLLYRGPVDPANWFGVRKGFPNLGYIQNHLQVLLLLVFEAIVYRRQEHYRRQHQLAPLPAQAVFASGTRQQLDQDLLGCLKYFINFFFYKFGLEICFLMAVNVIGQRMNFLVTLHGCWLVAILTRRHRQAIARLWPNYCLFLALFLLYQYLLCLGMPPALCIDYPWRWSRAVPMNSALIKWLYLPDFFRAPNSTNLISDFLLLLCASQQWQVFSAERTEEWQRMAGVNTDRLEPLRGEPNPVPNFIHCRSYLDMLKVAVFRYLFWLVLVVVFVTGATRISIFGLGYLLACFYLLLFGTALLQRDTRARLVLWDCLILYNVTVIISKNMLSLLACVFVEQMQTGFCWVIQLFSLVCTVKGYYDPKEMMDRDQDCLLPVEEAGIIWDSVCFFFLLLQRRVFLSHYYLHVRADLQATALLASRGFALYNAANLKSIDFHRRIEEKSLAQLKRQMERIRAKQEKHRQGRVDRSRPQDTLGPKDPGLEPGPDSPGGSSPPRRQWWRPWLDHATVIHSGDYFLFESDSEEEEEAVPEDPRPSAQSAFQLAYQAWVTNAQAVLRRRQQEQEQARQEQAGQLPTGGGPSQEVEPAEGPEEAAAGRSHVVQRVLSTAQFLWMLGQALVDELTRWLQEFTRHHGTMSDVLRAERYLLTQELLQGGEVHRGVLDQLYTSQAEATLPGPTEAPNAPSTVSSGLGAEEPLSSMTDDMGSPLSTGYHTRSGSEEAVTDPGEREAGASLYQGLMRTASELLLDRRLRIPELEEAELFAEGQGRALRLLRAVYQCVAAHSELLCYFIIILNHMVTASAGSLVLPVLVFLWAMLSIPRPSKRFWMTAIVFTEIAVVVKYLFQFGFFPWNSHVVLRRYENKPYFPPRILGLEKTDGYIKYDLVQLMALFFHRSQLLCYGLWDHEEDSPSKEHDKSGEEEQGAEEGPGVPAATTEDHIQVEARVGPTDGTPEPQVELRPRDTRRISLRFRRRKKEGPARKGAAAIEAEDREEEEGEEEKEAPTGREKRPSRSGGRVRAAGRRLQGFCLSLAQGTYRPLRRFFHDILHTKYRAATDVYALMFLADVVDFIIIIFGFWAFGKHSAATDITSSLSDDQVPEAFLVMLLIQFSTMVVDRALYLRKTVLGKLAFQVALVLAIHLWMFFILPAVTERMFNQNVVAQLWYFVKCIYFALSAYQIRCGYPTRILGNFLTKKYNHLNLFLFQGFRLVPFLVELRAVMDWVWTDTTLSLSSWMCVEDIYANIFIIKCSRETEKKYPQPKGQKKKKIVKYGMGGLIILFLIAIIWFPLLFMSLVRSVVGVVNQPIDVTVTLKLGGYEPLFTMSAQQPSIIPFTAQAYEELSRQFDPQPLAMQFISQYSPEDIVTAQIEGSSGALWRISPPSRAQMKRELYNGTADITLRFTWNFQRDLAKGGTVEYANEKHMLALAPNSTARRQLASLLEGTSDQSVVIPNLFPKYIRAPNGPEANPVKQLQPNEEADYLGVRIQLRREQGAGATGFLEWWVIELQECRTDCNLLPMVIFSDKVSPPSLGFLAGYGIMGLYVSIVLVIGKFVRGFFSEISHSIMFEELPCVDRILKLCQDIFLVRETRELELEEELYAKLIFLYRSPETMIKWTREKE